European Patent Specification EP 4 196 608 B1, published October 23, 2024. Title: NEGATIVELY CHARGED NANOPORES, POSITIVELY CHARGED NUCLEOTIDE OLIGOPHOSPHATES, AND USES THEREOF. Applicant: Roche Sequencing Solutions, Inc. Roche Diagnostics GmbH F. Hoffmann-La Roche AG. The sequence listing filed with the application follows.

SEQUENCE LISTING (243 sequences)

SEQ ID NO: 1 - protein, 305 aa, Staphylococcus aureus
ADSDINIKTGTTDIGSNTTVKTGDLVTYDKENGMHKKVFYSFIDDKNHNKKLLVIRTKGTIAGQYRVYSEEGANKSGLAWPSAFKVQLQLPDNEVAQISDYYPRNSIDTKEYMSTLTYGFNGNVTGDDTGKIGGLIGANVSIGHTLKYVQPDFKTILESPTDKKVGWKVIFNNMVNQNWGPYDRDSWNPVYGNQLFMKTRNGSMKAADNFLDPNKASSLLSSGFSPDFATVITMDRKASKQQTNIDVIYERVRDDYQLHWTSTNWKGTNTKDKWTDRSSERYKIDWEKEEMTNGLSAWSHPQFEK

SEQ ID NO: 2 - protein, 4 aa, Artificial Sequence
  Tag repeat structure
KKPP

SEQ ID NO: 3 - protein, 5 aa, Artificial Sequence
  Tag repeat structure
KKPPP

SEQ ID NO: 4 - protein, 4 aa, Artificial Sequence
  Tag repeat structure
KKGG

SEQ ID NO: 5 - protein, 4 aa, Artificial Sequence
  Tag repeat structure
KKGP

SEQ ID NO: 6 - protein, 4 aa, Artificial Sequence
  Tag repeat structure
KGPP

SEQ ID NO: 7 - protein, 4 aa, Artificial Sequence
  Tag repeat structure
KAPP

SEQ ID NO: 8 - protein, 4 aa, Artificial Sequence
  Tag repeat structure
KAAA

SEQ ID NO: 9 - protein, 4 aa, Artificial Sequence
  Tag repeat structure
KFPP

SEQ ID NO: 10 - protein, 4 aa, Artificial Sequence
  Tag repeat structure
KHPP

SEQ ID NO: 11 - protein, 4 aa, Artificial Sequence
  Tag repeat structure
KLPP

SEQ ID NO: 12 - protein, 4 aa, Artificial Sequence
  Tag repeat structure
KQPP

SEQ ID NO: 13 - protein, 4 aa, Artificial Sequence
  Tag repeat structure
KSPP

SEQ ID NO: 14 - protein, 4 aa, Artificial Sequence
  Tag repeat structure
  MISC_FEATURE (1)..(2): These residues are epsilon-linked lysine
KKPP

SEQ ID NO: 15 - protein, 4 aa, Artificial Sequence
  Tag repeat structure
  misc_feature (1)..(2): K is epsilon-linked lysine
  misc_feature (3)..(3): X is 4-Benzyloxyproline (BnoP)
KKXP

SEQ ID NO: 16 - protein, 4 aa, Artificial Sequence
  Tag repeat structure
  MISC_FEATURE (1)..(2): X is 4-aminoproline (4Ap)
XXPP

SEQ ID NO: 17 - protein, 4 aa, Artificial Sequence
  Tag repeat structure
RRPP

SEQ ID NO: 18 - protein, 5 aa, Artificial Sequence
  Tag repeat structure
RRPPP

SEQ ID NO: 19 - protein, 4 aa, Artificial Sequence
  Tag repeat structure
  MISC_FEATURE (1)..(2): X is aminoethylglycine (Aeg)
XXPP

SEQ ID NO: 20 - protein, 319 aa, Staphylococcus aureus
MKTRIVSSVTTTLLLGSILMNPVAGAADSDINIKTGTTDIGSNTTVKTGDLVTYDKENGMHKKVFYSFIDDKNHNKKLLVIRTKGTIAGQYRVYSEEGANKSGLAWPSAFKVQLQLPDNEVAQISDYYPRNSIDTKEYMSTLTYGFNGNVTGDDTGKIGGLIGANVSIGHTLKYVQPDFKTILESPTDKKVGWKVIFNNMVNQNWGPYDRDSWNPVYGNQLFMKTRNGSMKAADNFLDPNKASSLLSSGFSPDFATVITMDRKASKQQTNIDVIYERVRDDYQLHWTSTNWKGTNTKDKWTDRSSERYKIDWEKEEMTN

SEQ ID NO: 21 - protein, 301 aa, Escherichia coli (strain K12)
MKKLLPCTALVMCAGMACAQAEERNDWHFNIGAMYEIENVEGYGEDMDGLAEPSVYFNAANGPWRIALAYYQEGPVDYSAGKRGTWFDRPELEVHYQFLENDDFSFGLTGGFRNYGYHYVDEPGKDTANMQRWKIAPDWDVKLTDDLRFNGWLSMYKFANDLNTTGYADTRVETETGLQYTFNETVALRVNYYLERGFNMDDSRNNGEFSTQEIRAYLPLTLGNHSVTPYTRIGLDRWSNWDWQDDIEREGHDFNRVGLFYGYDFQNGLSVSLEYAFEWQDHDEGDSDKFHYAGVGVNYSF

SEQ ID NO: 22 - protein, 211 aa, Mycobacterium smegmatis (strain ATCC 70084 / mc(2)155)
MKAISRVLIAMVAAIAALFTSTGTSHAGLDNELSLVDGQDRTLTVQQWDTFLNGVFPLDRNRLTREWFHSGRAKYIVAGPGADEFEGTLELGYQIGFPWSLGVGINFSYTTPNILIDDGDITAPPFGLNSVITPNLFPGVSISADLGNGPGIQEVATFSVDVSGAEGGVAVSNAHGTVTGAAGGVLLRPFARLIASTGDSVTTYGEPWNMN

SEQ ID NO: 23 - protein, 280 aa, Escherichia coli (strain K12)
EERNDWHFNIGAMYEIENVEGYGEDMDGLAEPSVYFNAANGPWRIALAYYQEGPVDYSAGKRGTWFDRPELEVHYQFLENDDFSFGLTGGFRNYGYHYVDEPGKDTANMQRWKIAPDWDVKLTDDLRFNGWLSMYKFANDLNTTGYADTRVETETGLQYTFNETVALRVNYYLERGFNMDDSRNNGEFSTQEIRAYLPLTLGNHSVTPYTRIGLDRWSNWDWQDDIEREGHDFNRVGLFYGYDFQNGLSVSLEYAFEWQDHDEGDSDKFHYAGVGVNYSF

SEQ ID NO: 24 - protein, 268 aa, Artificial Sequence
  OmpG Variant
EERNDWHFNIGAMYEIENVEGYGEDMDGLAEPSVYFNAANGPWRIALAYYQEGPVDYSAGKRGTWFDRPELEVHYQFLENDDFSFGLTGGFRNYGYHYVDEPGKDTANMQRWKIAPDWDVKLTDDLRFNGWLSMYKFANDLNTTGYADTRVETETGLQYTFNETVALRVNYYLERGFNMDDSRNNGEFSTQEIRAYLPLTLGNHSVTPYTRIGLDRAGHDFNRVGLFYGYDFQNGLSVSLEYAFEWQDHDEGDSDKFHYAGVGVNYSF

SEQ ID NO: 25 - protein, 279 aa, Artificial Sequence
  OmpG Variant
EERNDWHFNIGAMYEIENVEGYGEDMDGLAEPSVYFNAANGPWRIALAYYQEGPVDYSAGKRGTWFDRPELEVHYQFLENDDFSFGLTGGFRNYGYHYVDEPGKDTANMQRWKIAPDWDVKLTDDLRFNGWLSMYKFANDLNTTGYADTRVETETGLQYTFNETVALRVNYYLERGFNMDDSRNNGEFSTQEIRAYLPLTLGNHSVTPYTRIGLRWSNWDWQDDIERECHDFNRVGLFYGYDFQNGLSVSLEYAFEWQDHCEGDSDKFHYAGVGVNYSF

SEQ ID NO: 26 - protein, 280 aa, Artificial Sequence
  OmpG Variant
EERNDWHFNIGAMYEIENVEGYGEDMDGLAEPSVYFNAANGPWRIALAYYQEGPVDYSAGKRGTWFDRPELEVHYQFLENDDFSFGLTGGFRNYGYHYVDEPGKDTANMQRWKIAPDWDVKLTDDLRFNGWLSMYKFANDLNTTGYADTRVETETGLQYTFNETVALRVNYYLERGFNMDDSRNNGEFSTQEIRAYLPLTLGNHSVTPYTRIGLDRWSNWDWQDDCEREGHDFNRVGLFYGYDFQNGLSVSLEYAFEWQDHDEGDSDKFHYAGVGVNYSF

SEQ ID NO: 27 - protein, 267 aa, Artificial Sequence
  OmpG Variant
EERNDWHFNIGAMYEIENVEGYGEDMDGLAEPSVYFNAANGPWRIALAYYQEGPVDYSAGKRGTWFDRPELEVHYQFLENDDFSFGLTGGFRNYGYHYVDEPGKDTANMQRWKIAPDWDVKLTDDLRFNGWLSMYKFANDLNTTGYADTRVETETGLQYTFNETVALRVNYYLERGFNMDDSRNNGEFSTQEIRAYLPLTLGNHSVTPYTRIGLRAGHDFNRVGLFYGYDFQNGLSVSLEYAFEWQDHDEGDSDKFHYAGVGVNYSF

SEQ ID NO: 28 - protein, 279 aa, Artificial Sequence
  OmpG Variant
EERNDWHFNIGAMYEIENVEGYGEDMDGLAEPSVYFNAANGPWRIALAYYQEGPVDYSAGKRGTWFDRPELEVHYQFLENDDFSFGLTGGFRNYGYHYVDEPGKDTANMQRWKIAPDWDVKLTDDLRFNGWLSMYKFANDLNTTGYADTRVETETGLQYTFNETVALRVNYYLERGFNMDDSRNNGEFSTQEIRAYLPLTLGNHSVTPYTRIGLRWSNWDWQDDCEREGHDFNRVGLFYGYDFQNGLSVSLEYAFEWQDHDEGDSDKFHYAGVGVNYSF

SEQ ID NO: 29 - protein, 184 aa, Mycobacteria Smegmatis
GLDNELSLVDGQDRTLTVQQWDTFLNGVFPLDRNRLTREWFHSGRAKYIVAGPGADEFEGTLELGYQIGFPWSLGVGINFSYTTPNILIDDGDITAPPFGLNSVITPNLFPGVSISADLGNGPGIQEVATFSVDVSGAEGGVAVSNAHGTVTGAAGGVLLRPFARLIASTGDSVTTYGEPWNMN

SEQ ID NO: 30 - protein, 739 aa, Artificial Sequence
  His-tagged Pol6
MHHHHHHHHSGGSDKHTQYVKEHSFNYDEYKKANFDKIECLIFDTESCTNYENDNTGARVYGWGLGVTRNHNMIYGQNLNQFWEVCQNIFNDWYHDNKHTIKITKTKKGFPKRKYIKFPIAVHNLGWDVEFLKYSLVENGFNYDKGLLKTVFSKGAPYQTVTDVEEPKTFHIVQNNNIVYGCNVYMDKFFEVENKDGSTTEIGLCLDFFDSYKIITCAESQFHNYVHDVDPMFYKMGEEYDYDTWRSPTHKQTTLELRYQYNDIYMLREVIEQFYIDGLCGGELPLTGMRTASSIAFNVLKKMTFGEEKTEEGYINYFELDKKTKFEFLRKRIEMESYTGGYTHANHKAVGKTINKIGCSLDINSSYPSQMAYKVFPYGKPVRKTWGRKPKTEKNEVYLIEVGFDFVEPKHEEYALDIFKIGAVNSKALSPITGAVSGQEYFCTNIKDGKAIPVYKELKDTKLTTNYNVVLTSVEYEFWIKHFNFGVFKKDEYDCFEVDNLEFTGLKIGSILYYKAEKGKFKPYVDHFTKMKVENKKLGNKPLTNQAKLILNGAYGKFGTKQNKEEKDLIMDKNGLLTFTGSVTEYEGKEFYRPYASFVTAYGRLQLWNAIIYAVGVENFLYCDTDSIYCNREVNSLIEDMNAIGETIDKTILGKWDVEHVFDKFKVLGQKKYMYHDCKEDKTDLKCCGLPSDARKIIIGQGFDEFYLGKNVEGKKQRKKVIGGCLLLDTLFTIKKIMF

SEQ ID NO: 31 - protein, 305 aa, Artificial Sequence
  aHL variant
DDSDINIKTGTTDIGSNTTVKTGDLVTYDKENGMGKKVFYSFIDDKNHNKKLLVIRTKGTIAGQYRVYSEEGANKSGLAWPSAFKVQLQLPDNEVAQISDYYPRNSIDTKEYMSTLTYGFNGNVTGDDTGKIGGLIGANVSIGATLKYVQPDFKTILESPTDKKVGWKVIFNNMVNQNWGPYDRDSWNPVYGNQLFMKTRNGSMKAADNFLDPNKASSLLSSGFSPDFATVITMDRKASKQQTNIDVIYERVRDDYQLHWTSTNWKGTNTKDKWTDRSSERYKIDWEKEEMTNGLSAWSHPQFEK

SEQ ID NO: 32 - protein, 305 aa, Artificial Sequence
  aHL variant
ADSDINIDTGTTDIGSNTTVKTGDLVTYDKENGMGKKVFYSFIDDKNHNKKLLVIRTKGTIAGQYRVYSEEGANKSGLAWPSAFKVQLQLPDNEVAQISDYYPRNSIDTKEYMSTLTYGFNGNVTGDDTGKIGGLIGANVSIGATLKYVQPDFKTILESPTDKKVGWKVIFNNMVNQNWGPYDRDSWNPVYGNQLFMKTRNGSMKAADNFLDPNKASSLLSSGFSPDFATVITMDRKASKQQTNIDVIYERVRDDYQLHWTSTNWKGTNTKDKWTDRSSERYKIDWEKEEMTNGLSAWSHPQFEK

SEQ ID NO: 33 - protein, 305 aa, Artificial Sequence
  aHL variant
ADSDINIKTGTTDIGSNTTVKTGDLVTYDKENGMLKKVFYSFIDDDNHNKKLLVIRTKGTIAGQYRVYSEEGANKSGLAWPSAFKVQLQLPDNEVAQISDYYPRNSIDTKEYMSTLTYGFNGNVTGDDTGKIGGLIGANVSIGHTLKYVQPDFKTILESPTDKKVGWKVIFNNMVNQNWGPYDRDSWNPVYGNQLFMKTRNGSMKAADNFLDPNKASSLLSSGFSPDFATVITMDRKASKQQTNIDVIYERVRDDYQLHWTSTNWKGTNTKDKWTDRSSERYKIDWEKEEMTNGLSAWSHPQFEK

SEQ ID NO: 34 - protein, 305 aa, Artificial Sequence
  aHL variant
ADSDINIKTGTTDIGSNTTVKTGDLVTYDKENGMGKKVFYSFIDDKDHNKKLLVIRTKGTIAGQYRVYSEEGANKSGLAWPSAFKVQLQLPDNEVAQISDYYPRNSIDTKEYMSTLTYGFNGNVTGDDTGKIGGLIGANVSIGATLKYDQPDFKTILESPTDKKVGWKVIFNNMVNQNWGPYDRDSWNPVYGNQLFMKTRNGSMKAADNFLDPNKASSLLSSGFSPDFATVITMDRKASKQQTNIDVIYERVRDDYQLHWTSTNWKGTNTKDKWTDRSSERYKIDWEKEEMTNGLSAWSHPQFEK

SEQ ID NO: 35 - protein, 305 aa, Artificial Sequence
  aHL variant
DDSDINIDTGTTDIGSNTTVKTGDLVTYDKENGMGKKVFYSFIDDKDHNKKLLVIRTKGTIAGQYRVYSEEGANKSGLAWPSAFKVQLQLPDNEVAQISDYYPRNSIDTKEYMSTLTYGFNGNVTGDDTGKIGGLIGANVSIGATLKYDQPDFKTILESPTDKKVGWKVIFNNMVNQNWGPYDRDSWNPVYGNQLFMKTRNGSMKAADNFLDPNKASSLLSSGFSPDFATVITMDRKASKQQTNIDVIYERVRDDYQLHWTSTNWKGTNTKDKWTDRSSERYKIDWEKEEMTNGLSAWSHPQFEK

SEQ ID NO: 36 - protein, 305 aa, Artificial Sequence
  aHL variant
ADSDINIDTGTTNIGSNTTVKTGDLVTYDKENGMGKKVFYSFIDDKNHNKKLLVIRTKGTIAGQYRVYSEEGANKSGLAWPSAFKVQLQLPDNEVAQISDYYPRNSIDTKEYMSTLTYGFNGNVTGDDTGKIGGLIGANVSIGATLKYVQPDFKTILESPTDKKVGWKVIFNNMVNQNWGPYDRDSWNPVYGNQLFMKTRNGSMKAADNFLDPNKASSLLSSGFSPDFATVITMDRKASKQQTNIDVIYERVRDDYQLHWTSTNWKGTNTKDKWTDRSSERYKIDWEKEEMTNGLSAWSHPQFEK

SEQ ID NO: 37 - protein, 305 aa, Artificial Sequence
  aHL variant
ADSDINIDTGTTNIGSNTTVKTGDLVTYDKENGMGKKVFYSFIDDKNHNKKLLVIRTKGTIAGQYRVYSEEGANKSGLAWPSAFKVQLQLPDNEVAQISDYYPRNSIDTKEYMSTLTYGFNGNVTGDDTGKIGGLIGANVSIGATLKYDQPDFKTILESPTDKKVGWKVIFNNMVNQNWGPYDRDSWNPVYGNQLFMKTRNGSMKAADNFLDPNKASSLLSSGFSPDFATVITMDRKASKQQTNIDVIYERVRDDYQLHWTSTNWKGTNTKDKWTDRSSERYKIDWEKEEMTNGLSAWSHPQFEK

SEQ ID NO: 38 - protein, 306 aa, Artificial Sequence
  aHL variant
DADSDINIKTGTTDIGSNTTVKTGDLVTYDKENGMGKKVFYSFIDDKNHNKKLLVIRTKGTIAGQYRVYSEEGANKSGLAWPSAFKVQLQLPDNEVAQISDYYPRNSIDTKEYMSTLTYGFNGNVTGDDTGKIGGLIGANVSIGATLKYVQPDFKTILESPTDKKVGWKVIFNNMVNQNWGPYDRDSWNPVYGNQLFMKTRNGSMKAADNFLDPNKASSLLSSGFSPDFATVITMDRKASKQQTNIDVIYERVRDDYQLHWTSTNWKGTNTKDKWTDRSSERYKIDWEKEEMTNGLSAWSHPQFEK

SEQ ID NO: 39 - protein, 306 aa, Artificial Sequence
  aHL variant
DDDSDINIKTGTTDIGSNTTVKTGDLVTYDKENGMGKKVFYSFIDDKNHNKKLLVIRTKGTIAGQYRVYSEEGANKSGLAWPSAFKVQLQLPDNEVAQISDYYPRNSIDTKEYMSTLTYGFNGNVTGDDTGKIGGLIGANVSIGATLKYVQPDFKTILESPTDKKVGWKVIFNNMVNQNWGPYDRDSWNPVYGNQLFMKTRNGSMKAADNFLDPNKASSLLSSGFSPDFATVITMDRKASKQQTNIDVIYERVRDDYQLHWTSTNWKGTNTKDKWTDRSSERYKIDWEKEEMTNGLSAWSHPQFEK

SEQ ID NO: 40 - protein, 306 aa, Artificial Sequence
  aHL variant
DADSDINIKTGTTDIGSNTTVKTGDLVTYDKENGMGKKVFYSFIDDKDHNKKLLVIRTKGTIAGQYRVYSEEGANKSGLAWPSAFKVQLQLPDNEVAQISDYYPRNSIDTKEYMSTLTYGFNGNVTGDDTGKIGGLIGANVSIGATLKYVQPDFKTILESPTDKKVGWKVIFNNMVNQNWGPYDRDSWNPVYGNQLFMKTRNGSMKAADNFLDPNKASSLLSSGFSPDFATVITMDRKASKQQTNIDVIYERVRDDYQLHWTSTNWKGTNTKDKWTDRSSERYKIDWEKEEMTNGLSAWSHPQFEK

SEQ ID NO: 41 - protein, 306 aa, Artificial Sequence
  aHL variant
DADSDINIDTGTTDIGSNTTVKTGDLVTYDKENGMGKKVFYSFIDDKNHNKKLLVIRTKGTIAGQYRVYSEEGANKSGLAWPSAFKVQLQLPDNEVAQISDYYPRNSIDTKEYMSTLTYGFNGNVTGDDTGKIGGLIGANVSIGATLKYVQPDFKTILESPTDKKVGWKVIFNNMVNQNWGPYDRDSWNPVYGNQLFMKTRNGSMKAADNFLDPNKASSLLSSGFSPDFATVITMDRKASKQQTNIDVIYERVRDDYQLHWTSTNWKGTNTKDKWTDRSSERYKIDWEKEEMTNGLSAWSHPQFEK

SEQ ID NO: 42 - protein, 306 aa, Artificial Sequence
  aHL variant
DDDSDINIDTGTTDIGSNTTVKTGDLVTYDKENGMGKKVFYSFIDDKNHNKKLLVIRTKGTIAGQYRVYSEEGANKSGLAWPSAFKVQLQLPDNEVAQISDYYPRNSIDTKEYMSTLTYGFNGNVTGDDTGKIGGLIGANVSIGATLKYVQPDFKTILESPTDKKVGWKVIFNNMVNQNWGPYDRDSWNPVYGNQLFMKTRNGSMKAADNFLDPNKASSLLSSGFSPDFATVITMDRKASKQQTNIDVIYERVRDDYQLHWTSTNWKGTNTKDKWTDRSSERYKIDWEKEEMTNGLSAWSHPQFEK

SEQ ID NO: 43 - protein, 305 aa, Artificial Sequence
  aHL variant
DDSDINIKTGTTDIGSNTTVKTGDLVTYDKENGMGKKVFYSFIDDKNHNKKLLVIRTKGTIAGQYRVYSEEGANKSGLAWPSAFKVQLQLPDNEVAQISDYYPRNSIDTKEYDSDLDYGFDGNVTGDDTGKIGGLIGANVSIGATLKYVQPDFKTILESPTDKKVGWKVIFNNMVNQNWGPYDRDSWNPVYGNQLFMKTRNGSMKAADNFLDPNKASSLLSSGFSPDFATVITMDRKASKQQTNIDVIYERVRDDYQLHWTSTNWKGTNTKDKWTDRSSERYKIDWEKEEMTNGLSAWSHPQFEK

SEQ ID NO: 44 - protein, 305 aa, Artificial Sequence
  aHL variant
DDDDINIKTDTTDIGSNTTVKTGDLVTYDKENGMGKKVFYSFIDDDNHNKKLLVIRTKGTIAGQYRVYSEEGANKSGLAWPSAFKVQLQLPDNEVAQISDYYPRNDIDTKEYMSTLTYGFNGNVTGDDTGKIGGLIGANVSIGATLKYVQPDFKTILESPTDKKVGWKVIFNNMVNQNWGPYDRDSWNPVYGNQLFMKTRNGSMKAADNFLDPNKASSLLSSGFSPDFATVITMDRKASKQQTNIDVIYERVRDDYQLHWTSTNWKGTNTKDKWTDRSSERYKIDWEKEEMTNGLSAWSHPQFEK

SEQ ID NO: 45 - protein, 305 aa, Artificial Sequence
  aHL variant
ADSDINIKTDTTDIGSNTTVKTGDLVTYDKENGMGKKVFYSFIDDKNHNKKLLVIRTKGTIAGQYRVYSEEGANKSGLAWPSAFKVQLQLPDNEVAQISDYYPRNSIDTKEYDSDLDYGFDGNVTGDDTGKIGGLIGANVSIGATLKYVQPDFKTILESPTDKKVGWKVIFNNMVNQNWGPYDRDSWNPVYGNQLFMKTRNGSMKAADNFLDPNKASSLLSSGFSPDFATVITMDRKASKQQTNIDVIYERVRDDYQLHWTSTNWKGTNTKDKWTDRSSERYKIDWEKEEMTNGLSAWSHPQFEK

SEQ ID NO: 46 - protein, 305 aa, Artificial Sequence; identical to SEQ ID NO: 36
  aHL variant

SEQ ID NO: 47 - protein, 305 aa, Artificial Sequence
  aHL variant
ADSDINIDTGTTNIGSNTTVKTGDLVTYDKENGMGKKVFYSFIDDKNHNKKLLVIRTKGTIAGQYRVYSEEGANKSGLAWPSAFKVQLQLPDNEVAQISDYYPRNSIDTKEYMSTLTYGFNGNVTGDDTGKIGGLIGANVSIGHTLKYDQPDFKTILESPTDKKVGWKVIFNNMVNQNWGPYDRDSWNPVYGNQLFMKTRNGSMKAADNFLDPNKASSLLSSGFSPDFATVITMDRKASKQQTNIDVIYERVRDDYQLHWTSTNWKGTNTKDKWTDRSSERYKIDWEKEEMTNGLSAWSHPQFEK

SEQ ID NO: 48 - protein, 306 aa, Artificial Sequence; identical to SEQ ID NO: 38
  aHL variant

SEQ ID NO: 49 - protein, 306 aa, Artificial Sequence; identical to SEQ ID NO: 39
  aHL variant

SEQ ID NO: 50 - protein, 306 aa, Artificial Sequence; identical to SEQ ID NO: 40
  aHL variant

SEQ ID NO: 51 - protein, 306 aa, Artificial Sequence; identical to SEQ ID NO: 41
  aHL variant

SEQ ID NO: 52 - protein, 306 aa, Artificial Sequence; identical to SEQ ID NO: 42
  aHL variant

SEQ ID NO: 53 - protein, 305 aa, Artificial Sequence
  aHL variant
ADSDINIKTGTTDIGSNTTVKTGDLVTYDKENGMGKKVFYSFIDDKNHNKKLLVIRTKGTIAGQYRVYSEEGANKSGLAWPSAFKVQLQLPDNEVAQISDYYPRNSIDTKAYDSDLDYGFDGNVTGDDTGKIGGLIGANVSIGATLAYVQPDFKTILESPTDKKVGWKVIFNNMVNQNWGPYDRDSWNPVYGNQLFMKTRNGSMKAADNFLDPNKASSLLSSGFSPDFATVITMDRKASKQQTNIDVIYERVRDDYQLHWTSTNWKGTNTKDKWTDRSSERYKIDWEKEEMTNGLSAWSHPQFEK

SEQ ID NO: 54 - protein, 305 aa, Artificial Sequence
  aHL variant
DDSDINIKDGTTDIGSNTTVKTGDLVTYDKENGMGKKVFYSFIDDKKHNKKLLVIRTKGTIAGQYRVYSEEGANKSGLAWPSAFKVQLQLPDNEVAQISDYYPRNSIDTKEYMSTLTYGFNGNVTGDDDDKIGGLIGANVSIGATLKYVQPDFKTILESPTDKKVGWKVIFNNMVNQNWGPYDRDSWNPVYGNQLFMKTRNGSMKAADNFLDPNKASSLLSSGFSPDFATVITMDRKASKQQTNIDVIYERVRDDYQLHWTSTNWKGTNTKDKWTDRSSERYKIDWEKEEMTNGLSAWSHPQFEK

SEQ ID NO: 55 - protein, 305 aa, Artificial Sequence
  aHL variant
DDSDINIKTGTTDIGSNTTVKTGDLVTYDKENGMGKKVFYSFIDDKKHNKKLLVIRTKGTIAGQYRVYSEEGANKSGLAWPSAFKVQLQLPDNEVAQISDYYPRNSIDTKEYMSTLTYGFNGNVTGDDDDKIGGLIGANVSIGATLKYVQPDFKTILESPTDKKVGWKVIFNNMVNQNWGPYDRDSWNPVYGNQLFMKTRNGSMKAADNFLDPNKASSLLSSGFSPDFATVITMDRKASKQQTNIDVIYERVRDDYQLHWTSTNWKGTNTKDKWTDRSSERYKIDWEKEEMTNGLSAWSHPQFEK

SEQ ID NO: 56 - protein, 305 aa, Artificial Sequence
  aHL variant
ADSDINIKTGTTDIGSNTTVKTGDLVTYDKENGMGKKVFYSFIDDKNHNKKLLVIRTKGTIAGQYRVYSEEGANKSGLAWPSAFKVQLQLPDNEVAQISDYYPRNSIDTKEYDSDLDYGFDGNVTGDDTGKIGGLIGANVSIGHTLKYVQPDFKTILESPTDKKVGWKVIFNNMVNQNWGPYDRDSWNPVYGNQLFMKTRNGSMKAADNFLDPNKASSLLSSGFSPDFATVITMDRKASKQQTNIDVIYERVRDDYQLHWTSTNWKGTNTKDKWTDRSSERYKIDWEKEEMTNGLSAWSHPQFEK

SEQ ID NO: 57 - protein, 305 aa, Artificial Sequence
  aHL variant
DDSDINIKTGTTDIGSNTTVKTGDLVTYDKENGMGKKVFYSFIDDKKHNKKLLVIRTKGTIAGQYRVYSEEGANKSGLAWPSAFKVQLQLPDNEVAQISDYYPRNSIDTKEYMSTLTYGFNGNVTGDDDDDIGGLIGANVSIGATLDYVQPDFKTILESPTDKKVGWKVIFNNMVNQNWGPYDRDSWNPVYGNQLFMKTRNGSMKAADNFLDPNKASSLLSSGFSPDFATVITMDRKASKQQTNIDVIYERVRDDYQLHWTSTNWKGTNTKDKWTDRSSERYKIDWEKEEMTNGLSAWSHPQFEK

SEQ ID NO: 58 - protein, 305 aa, Artificial Sequence
  aHL variant
DDSDINIKTGTTDIGSDTTVKTGDLVTYDKENGMGKKVFYSFIDDKNHNKKLLVIRTKGTIAGQYRVYSEEGANKSGLAWPSAFKVQLQLPDNEVAQISDYYPRNSIDTKEYMSTLTYGFNGNVTGDDTGDIGGLIGANVSIGATLKYVQPDFKTILESPTDKKVGWKVIFNNMVNQNWGPYDRDSWNPVYGNQLFMKTRNGSMKAADNFLDPNKASSLLSSGFSPDFATVITMDRKASKQQTNIDVIYERVRDDYQLHWTSTNWKGTNTKDKWTDRSSERYKIDWEKEEMTNGLSAWSHPQFEK

SEQ ID NO: 59 - protein, 305 aa, Artificial Sequence
  aHL variant
DDSDINIKTGTTDIGSNTTVKTGDLVTYDKENGMHKKVFYSFIDDKNHNKKLLVIRTKGTIAGQYRVYSEEGANKSGLAWPSAFKVQLQLPDNEVAQISDYYPRNSIDTKEYMSTLTYGFNGNVTGDDTGDIGGLIGANVSIGHTLDYVQPDFKTILESPTDKKVGWKVIFNNMVNQNWGPYDRDSWNPVYGNQLFMKTRNGSMKAADNFLDPNKASSLLSSGFSPDFATVITMDRKASKQQTNIDVIYERVRDDYQLHWTSTNWKGTNTKDKWTDRSSERYKIDWEKEEMTNGLSAWSHPQFEK

SEQ ID NO: 60 - protein, 305 aa, Artificial Sequence
  aHL variant
ADSDINIKTGTTDIGSDTTVKTGDLVTYDKENGMGKKVFYSFIDDKKHNKKLLVIRTKGTIAGQYRVYSEEGANKSKLAWPSAFKVQLQLPDNEVAQISDYYPRNSIDTKAYASDLDYGFDGNVTGDKTGKIGGLIGANVSIGHTLAYVQPDFKTILESPTDKKVGWKVIFNKMVNQNWGPYDRDSWNPVYGNQLFMKTRNGSMKAADNFLDPNKASSLLSSGFSPDFATVITMDRKASKQQTNIDVIYERVRDDYQLHWTSTNWKGTNTKDKWTDRSSERYKIDWEKEEMTNGLSAWSHPQFEK

SEQ ID NO: 61 - protein, 305 aa, Artificial Sequence
  aHL variant
ADSDINIKTGTTDIGSDTTVKTGDLVTYDKENGMHKKVFYSFIDDKKHNKKLLVIRTKGTIAGQYRVYSEEGANKSKLAWPSAFKVQLQLPDNEVAQISDYYPRNSIDTKAYASDLDYGFDGNVTGDKTGKIGGLIGANVSIGHTLAYVQPDFKTILESPTDKKVGWKVIFNKMVNQNWGPYDRDSWNPVYGNQLFMKTRNGSMKAADNFLDPNKASSLLSSGFSPDFATVITMDRKASKQQTNIDVIYERVRDDYQLHWTSTNWKGTNTKDKWTDRSSERYKIDWEKEEMTNGLSAWSHPQFEK

SEQ ID NO: 62 - protein, 305 aa, Artificial Sequence
  aHL variant
DDSDINIKTGTTDIGSNTTVKTGDLVTYDKENGMLKKVFYSFIDDKNHNKKLLVIRTKGTIAGQYRVYSEEGANKSGLAWPSAFKVQLQLPDNEVAQISDYYPRNSIDTKEYMSTLTYGFNGNVTGDDTGDIGGLIGANVSIGHTLDYVQPDFKTILESPTDKKVGWKVIFNNMVNQNWGPYDRDSWNPVYGNQLFMKTRNGSMKAADNFLDPNKASSLLSSGFSPDFATVITMDRKASKQQTNIDVIYERVRDDYQLHWTSTNWKGTNTKDKWTDRSSERYKIDWEKEEMTNGLSAWSHPQFEK

SEQ ID NO: 63 - protein, 305 aa, Artificial Sequence
  aHL variant
DDSDINIDTGTTDIGSNTTVKTGDLVTYDKENGMLKKVFYSFIDDKNHNKKLLVIRTKGTIAGQYRVYSEEGANKSGLAWPSAFKVQLQLPDNEVAQISDYYPRNSIDTKEYMSTLTYGFNGNVTGDDTGDIGGLIGANVSIGATLDYVQPDFKTILESPTDKKVGWKVIFNNMVNQNWGPYDRDSWNPVYGNQLFMKTRNGSMKAADNFLDPNKASSLLSSGFSPDFATVITMDRKASKQQTNIDVIYERVRDDYQLHWTSTNWKGTNTKDKWTDRSSERYKIDWEKEEMTNGLSAWSHPQFEK

SEQ ID NO: 64 - protein, 305 aa, Artificial Sequence
  aHL variant
DDSDINIKTGTTDIGSDTTVKTGDLVTYDKENGMLKKVFYSFIDDKNHNKKLLVIRTKGTIAGQYRVYSEEGANKSGLAWPSAFKVQLQLPDNEVAQISDYYPRNSIDTKEYMSTLTYGFNGNVTGDDTGDIGGLIGANVSIGATLDYVQPDFKTILESPTDKKVGWKVIFNNMVNQNWGPYDRDSWNPVYGNQLFMKTRNGSMKAADNFLDPNKASSLLSSGFSPDFATVITMDRKASKQQTNIDVIYERVRDDYQLHWTSTNWKGTNTKDKWTDRSSERYKIDWEKEEMTNGLSAWSHPQFEK

SEQ ID NO: 65 - protein, 305 aa, Artificial Sequence
  aHL variant
DDSDINIDTGTTDIGSNTTVKTGDLVTYDKENGMLKKVFYSFIDDKNHNKKLLVIRTKGTIAGQYRVYSEEGANKSGLAWPSAFKVQLQLPDNEVAQISDYYPRNSIDTKEYMSDLDYGFNGNVTGDDTGDIGGLIGANVSIGATLDYVQPDFKTILESPTDKKVGWKVIFNNMVNQNWGPYDRDSWNPVYGNQLFMKTRNGSMKAADNFLDPNKASSLLSSGFSPDFATVITMDRKASKQQTNIDVIYERVRDDYQLHWTSTNWKGTNTKDKWTDRSSERYKIDWEKEEMTNGLSAWSHPQFEK

SEQ ID NO: 66 - protein, 305 aa, Artificial Sequence
  aHL variant
ADSDINIKTGTTDIGSDTTVKTGDLVTYDKENGMLKKVFYSFIDDKDHNKKLLVIRTKGTIAGQYRVYSEEGANKSGLAWPSAFKVQLQLPDNEVAQISDYYPRNSIDTKAYDSDLDYGFDGNVTGDDTGKIGGLIGANVSIGHTLAYVQPDFKTILESPTDKKVGWKVIFNNMVNQNWGPYDRDSWNPVYGNQLFMKTRNGSMKAADNFLDPNKASSLLSSGFSPNFATVITMDRKASKQQTNIDVIYERVRDDYQLHWTSTNWKGTNTKDKWTDRSSERYKIDWEKEEMTNGLSAWSHPQFEK

SEQ ID NO: 67 - protein, 305 aa, Artificial Sequence
  aHL variant
ADSDINIDTGTTDIGSNTTVKTGDLVTYDKENGMLKKVFYSFIDDKDHNKKLLVIRTKGTIAGQYRVYSEEGANKSGLAWPSAFKVQLQLPDNEVAQISDYYPRNSIDTKAYDSDLDYGFDGNVTGDDTGKIGGLIGANVSIGHTLAYVQPDFKTILESPTDKKVGWKVIFNNMVNQNWGPYDRDSWNPVYGNQLFMKTRNGSMKAADNFLDPNKASSLLSSGFSPNFATVITMDRKASKQQTNIDVIYERVRDDYQLHWTSTNWKGTNTKDKWTDRSSERYKIDWEKEEMTNGLSAWSHPQFEK

SEQ ID NO: 68 - protein, 305 aa, Artificial Sequence
  aHL variant
DDSDINIKDGTTDIGSNTTVKTGDLVTYDKENGMLKKVFYSFIDDKNHNKKLLVIRTKGTIAGQYRVYSEEGANKSGLAWPSAFKVQLQLPDNEVAQISDYYPRNSIDTKEYMSTLTYGFNGNVTGDDTGDIGGLIGANVSIGATLDYVQPDFKTILESPTDKKVGWKVIFNNMVNQNWGPYDRDSWNPVYGNQLFMKTRNGSMKAADNFLDPNKASSLLSSGFSPDFATVITMDRKASKQQTNIDVIYERVRDDYQLHWTSTNWKGTNTKDKWTDRSSERYKIDWEKEEMTNGLSAWSHPQFEK

SEQ ID NO: 69 - protein, 305 aa, Artificial Sequence
  aHL variant
DDSDINIDTGTTDIGSNTTVKTGDLVTYDKENGMLKKVFYSFIDDKNHNKKLLVIRTKGTIAGQYRVYSEEGANKSGLAWPSAFKVQLQLPDNEVAQISDYYPRNSIDTKEYMSTLTYGFDGNVTGDDTGDIGGLIGANVSIGATLDYVQPDFKTILESPTDKKVGWKVIFNNMVNQNWGPYDRDSWNPVYGNQLFMKTRNGSMKAADNFLDPNKASSLLSSGFSPDFATVITMDRKASKQQTNIDVIYERVRDDYQLHWTSTNWKGTNTKDKWTDRSSERYKIDWEKEEMTNGLSAWSHPQFEK

SEQ ID NO: 70 - protein, 305 aa, Artificial Sequence
  aHL variant
DDSDINIDTGTTDIGSNTTVKTGDLVTYDKENGMLKKVFYSFIDDKNHNKKLLVIRTKGTIAGQYRVYSEEGANKSGLAWPSAFKVQLQLPDNEVAQISDYYPRNSIDTKEYMSTLTYGFNGDVTGDDTGDIGGLIGANVSIGATLDYVQPDFKTILESPTDKKVGWKVIFNNMVNQNWGPYDRDSWNPVYGNQLFMKTRNGSMKAADNFLDPNKASSLLSSGFSPDFATVITMDRKASKQQTNIDVIYERVRDDYQLHWTSTNWKGTNTKDKWTDRSSERYKIDWEKEEMTNGLSAWSHPQFEK

SEQ ID NO: 71 - protein, 305 aa, Artificial Sequence
  aHL variant
DDSDINIKTGTTDIGSDTTVKTGDLVTYDKENGMLKKVFYSFIDDKNHNKKLLVIRTKGTIAGQYRVYSEEGANKSGLAWPSAFKVQLQLPDNEVAQISDYYPRNSIDTKEYMSTLTYGFDGNVTGDDTGDIGGLIGANVSIGATLDYVQPDFKTILESPTDKKVGWKVIFNNMVNQNWGPYDRDSWNPVYGNQLFMKTRNGSMKAADNFLDPNKASSLLSSGFSPDFATVITMDRKASKQQTNIDVIYERVRDDYQLHWTSTNWKGTNTKDKWTDRSSERYKIDWEKEEMTNGLSAWSHPQFEK

SEQ ID NO: 72 - protein, 305 aa, Artificial Sequence
  aHL variant
DDSDINIKTGTTDIGSDTTVKTGDLVTYDKENGMLKKVFYSFIDDKNHNKKLLVIRTKGTIAGQYRVYSEEGANKSGLAWPSAFKVQLQLPDNEVAQISDYYPRNSIDTKEYMSTLTYGFNGDVTGDDTGDIGGLIGANVSIGATLDYVQPDFKTILESPTDKKVGWKVIFNNMVNQNWGPYDRDSWNPVYGNQLFMKTRNGSMKAADNFLDPNKASSLLSSGFSPDFATVITMDRKASKQQTNIDVIYERVRDDYQLHWTSTNWKGTNTKDKWTDRSSERYKIDWEKEEMTNGLSAWSHPQFEK

SEQ ID NO: 73 - protein, 305 aa, Artificial Sequence
  aHL variant
DDSDINIKTGTTDIGSDTTVKTGDLVTYDKENGMLKKVFYSFIDDKDHNKKLLVIRTKGTIAGQYRVYSEEGANKSGLAWPSAFKVQLQLPDNEVAQISDYYPRNSIDTKAYDSDLDYGFDGNVTGDDTGKIGGLIGANVSIGHTLAYVQPDFKTILESPTDKKVGWKVIFNNMVNQNWGPYDRDSWNPVYGNQLFMKTRNGSMKAADNFLDPNKASSLLSSGFSPNFATVITMDRKASKQQTNIDVIYERVRDDYQLHWTSTNWKGTNTKDKWTDRSSERYKIDWEKEEMTNGLSAWSHPQFEK

SEQ ID NO: 74 - protein, 305 aa, Artificial Sequence
  aHL variant
ADSDINIKTGTTDIGSDTTVKTGDLVTYDKENGMLKKVFYSFIDDKDHNKKLLVIRTKGTIAGQYRVYSEEGANKSGLAWPSAFKVQLQLPDNEVAQISDYYPRNSIDTKEYDSDLDYGFDGNVTGDDTGKIGGLIGANVSIGHTLAYVQPDFKTILESPTDKKVGWKVIFNNMVNQNWGPYDRDSWNPVYGNQLFMKTRNGSMKAADNFLDPNKASSLLSSGFSPNFATVITMDRKASKQQTNIDVIYERVRDDYQLHWTSTNWKGTNTKDKWTDRSSERYKIDWEKEEMTNGLSAWSHPQFEK

SEQ ID NO: 75 - protein, 305 aa, Artificial Sequence
  aHL variant
ADSDINIDDGTTNIGSNTTVKTGDLVTYDKENGMGKKVFYSFIDDKNHNKKLLVIRTKGTIAGQYRVYSEEGANKSGLAWPSAFKVQLQLPDNEVAQISDYYPRNSIDTKEYMSTLTYGFNGNVTGDDTGKIGGLIGANVSIGHTLKYVQPDFKTILESPTDKKVGWKVIFNNMVNQNWGPYDRDSWNPVYGNQLFMKTRNGSMKAADNFLDPNKASSLLSSGFSPDFATVITMDRKASKQQTNIDVIYERVRDDYQLHWTSTNWKGTNTKDKWTDRSSERYKIDWEKEEMTNGLSAWSHPQFEK

SEQ ID NO: 76 - protein, 305 aa, Artificial Sequence
  aHL variant
ADSDINIDTGTTNIGSNTTVKTGDLVTYDKENGMGKKVFYSFIDDKNHNKKLLVIRTKGTIAGQYRVYSEEGANKSGLAWPSAFKVQLQLPDNEVAQISDYYPRNDIDTKEYMSTLTYGFNGNVTGDDTGKIGGLIGANVSIGHTLKYVQPDFKTILESPTDKKVGWKVIFNNMVNQNWGPYDRDSWNPVYGNQLFMKTRNGSMKAADNFLDPNKASSLLSSGFSPDFATVITMDRKASKQQTNIDVIYERVRDDYQLHWTSTNWKGTNTKDKWTDRSSERYKIDWEKEEMTNGLSAWSHPQFEK

SEQ ID NO: 77 - protein, 305 aa, Artificial Sequence
  aHL variant
ADDDINIDTGTTNIGSNTTVKTGDLVTYDKENGMGKKVFYSFIDDKNHNKKLLVIRTKGTIAGQYRVYSEEGANKSGLAWPSAFKVQLQLPDNEVAQISDYYPRNSIDTKEYMSTLTYGFNGNVTGDDTGKIGGLIGANVSIGHTLKYVQPDFKTILESPTDKKVGWKVIFNNMVNQNWGPYDRDSWNPVYGNQLFMKTRNGSMKAADNFLDPNKASSLLSSGFSPDFATVITMDRKASKQQTNIDVIYERVRDDYQLHWTSTNWKGTNTKDKWTDRSSERYKIDWEKEEMTNGLSAWSHPQFEK

SEQ ID NO: 78 - protein, 305 aa, Artificial Sequence
  aHL variant
ADSDINIDTGTTNIGSDTTVKTGDLVTYDKENGMGKKVFYSFIDDKNHNKKLLVIRTKGTIAGQYRVYSEEGANKSGLAWPSAFKVQLQLPDNEVAQISDYYPRNSIDTKEYMSTLTYGFNGNVTGDDTGKIGGLIGANVSIGHTLKYVQPDFKTILESPTDKKVGWKVIFNNMVNQNWGPYDRDSWNPVYGNQLFMKTRNGSMKAADNFLDPNKASSLLSSGFSPDFATVITMDRKASKQQTNIDVIYERVRDDYQLHWTSTNWKGTNTKDKWTDRSSERYKIDWEKEEMTNGLSAWSHPQFEK

SEQ ID NO: 79 - protein, 305 aa, Artificial Sequence
  aHL variant
ADSDINIDTGTTNIGSNTTVKTGDLVTYDKENGMGKKVFYSFIDDKNHNKKLLVIRTKGTIAGQYRVYSEEGANKSGLAWPSAFKVQLQLPDNEVAQISDYYPRNSIDTKEYMSTLTYGFNGNVTGDDTGKIGGLIGANVSIGHTLKYVQPDFKTILESPTDKKVGWKVIFNNMVNQNWGPYDRDSWNPVYGNQLFMKTRNGSMKAADNFLDPNKASSLLSSGFSPDFATVITMDRKADKQQTNIDVIYERVRDDYQLHWTSTNWKGTNTKDKWTDRSSERYKIDWEKEEMTNGLSAWSHPQFEK

SEQ ID NO: 80 - protein, 305 aa, Artificial Sequence
  aHL variant
ADSDINIDTGTTNIGSNTTVKTGDLVTYDKENGMGKKVFYSFIDDKDHNKKLLVIRTKGTIAGQYRVYSEEGANKSGLAWPSAFKVQLQLPDNEVAQISDYYPRNSIDTKEYMSTLTYGFNGNVTGDDTGKIGGLIGANVSIGHTLKYVQPDFKTILESPTDKKVGWKVIFNNMVNQNWGPYDRDSWNPVYGNQLFMKTRNGSMKAADNFLDPNKASSLLSSGFSPDFATVITMDRKASKQQTNIDVIYERVRDDYQLHWTSTNWKGTNTKDKWTDRSSERYKIDWEKEEMTNGLSAWSHPQFEK

SEQ ID NO: 81 - protein, 305 aa, Artificial Sequence
  aHL variant
ADSDINIDTGTTNIGSNTTVKTGDLVTYDKENGMGKKVFYSFIDDDNHNKKLLVIRTKGTIAGQYRVYSEEGANKSGLAWPSAFKVQLQLPDNEVAQISDYYPRNSIDTKEYMSTLTYGFNGNVTGDDTGKIGGLIGANVSIGHTLKYVQPDFKTILESPTDKKVGWKVIFNNMVNQNWGPYDRDSWNPVYGNQLFMKTRNGSMKAADNFLDPNKASSLLSSGFSPDFATVITMDRKASKQQTNIDVIYERVRDDYQLHWTSTNWKGTNTKDKWTDRSSERYKIDWEKEEMTNGLSAWSHPQFEK

SEQ ID NO: 82 - protein, 305 aa, Artificial Sequence
  aHL variant
ADSDINIDTGTTNIGSNTTVKTGDLVTYDKENGMGKKVFYSFIDDKNHNKKLLVIRTKGTIAGQYRVYSEEGANKSGLAWPSAFKVQLQLPDNEVAQISDYYPRNSIDTKEYDSTLTYGFNGNVTGDDTGKIGGLIGANVSIGHTLKYVQPDFKTILESPTDKKVGWKVIFNNMVNQNWGPYDRDSWNPVYGNQLFMKTRNGSMKAADNFLDPNKASSLLSSGFSPDFATVITMDRKASKQQTNIDVIYERVRDDYQLHWTSTNWKGTNTKDKWTDRSSERYKIDWEKEEMTNGLSAWSHPQFEK

SEQ ID NO: 83 - protein, 305 aa, Artificial Sequence
  aHL variant
ADSDINIDTGTTNIGSNTTVKTGDLVTYDKENGMGKKVFYSFIDDKNHNKKLLVIRTKGTIAGQYRVYSEEGANKSGLAWPSAFKVQLQLPDNEVAQISDYYPRNSIDTKEYMSDLTYGFNGNVTGDDTGKIGGLIGANVSIGHTLKYVQPDFKTILESPTDKKVGWKVIFNNMVNQNWGPYDRDSWNPVYGNQLFMKTRNGSMKAADNFLDPNKASSLLSSGFSPDFATVITMDRKASKQQTNIDVIYERVRDDYQLHWTSTNWKGTNTKDKWTDRSSERYKIDWEKEEMTNGLSAWSHPQFEK

SEQ ID NO: 84 - protein, 305 aa, Artificial Sequence
  aHL variant
ADSDINIDTGTTNIGSNTTVKTGDLVTYDKENGMGKKVFYSFIDDKNHNKKLLVIRTKGTIAGQYRVYSEEGANKSGLAWPSAFKVQLQLPDNEVAQISDYYPRNSIDTKEYMSTLDYGFNGNVTGDDTGKIGGLIGANVSIGHTLKYVQPDFKTILESPTDKKVGWKVIFNNMVNQNWGPYDRDSWNPVYGNQLFMKTRNGSMKAADNFLDPNKASSLLSSGFSPDFATVITMDRKASKQQTNIDVIYERVRDDYQLHWTSTNWKGTNTKDKWTDRSSERYKIDWEKEEMTNGLSAWSHPQFEK

SEQ ID NO: 85 - protein, 305 aa, Artificial Sequence
  aHL variant
ADSDINIDTGTTNIGSNTTVKTGDLVTYDKENGMGKKVFYSFIDDKNHNKKLLVIRTKGTIAGQYRVYSEEGANKSGLAWPSAFKVQLQLPDNEVAQISDYYPRNSIDTKEYMSTLTYGFDGNVTGDDTGKIGGLIGANVSIGHTLKYVQPDFKTILESPTDKKVGWKVIFNNMVNQNWGPYDRDSWNPVYGNQLFMKTRNGSMKAADNFLDPNKASSLLSSGFSPDFATVITMDRKASKQQTNIDVIYERVRDDYQLHWTSTNWKGTNTKDKWTDRSSERYKIDWEKEEMTNGLSAWSHPQFEK

SEQ ID NO: 86 - protein, 305 aa, Artificial Sequence
  aHL variant
ADSDINIDTGTTNIGSNTTVKTGDLVTYDKENGMGKKVFYSFIDDKNHNKKLLVIRTKGTIAGQYRVYSEEGANKSGLAWPSAFKVQLQLPDNEVAQISDYYPRNSIDTKEYMSTLTYGFNGNVTGDDDGKIGGLIGANVSIGHTLKYVQPDFKTILESPTDKKVGWKVIFNNMVNQNWGPYDRDSWNPVYGNQLFMKTRNGSMKAADNFLDPNKASSLLSSGFSPDFATVITMDRKASKQQTNIDVIYERVRDDYQLHWTSTNWKGTNTKDKWTDRSSERYKIDWEKEEMTNGLSAWSHPQFEK

SEQ ID NO: 87 - protein, 305 aa, Artificial Sequence
  aHL variant
ADSDINIDTGTTNIGSNTTVKTGDLVTYDKENGMGKKVFYSFIDDKNHNKKLLVIRTKGTIAGQYRVYSEEGANKSGLAWPSAFKVQLQLPDNEVAQISDYYPRNSIDTKEYMSTLTYGFNGNVTGDDTDKIGGLIGANVSIGHTLKYVQPDFKTILESPTDKKVGWKVIFNNMVNQNWGPYDRDSWNPVYGNQLFMKTRNGSMKAADNFLDPNKASSLLSSGFSPDFATVITMDRKASKQQTNIDVIYERVRDDYQLHWTSTNWKGTNTKDKWTDRSSERYKIDWEKEEMTNGLSAWSHPQFEK

SEQ ID NO: 88 - protein, 305 aa, Artificial Sequence
  aHL variant
ADSDINIDTGTTNIGSNTTVKTGDLVTYDKENGMGKKVFYSFIDDKNHNKKLLVIRTKGTIAGQYRVYSEEGANKSGLAWPSAFKVQLQLPDNEVAQISDYYPRNSIDTKEYMSTLTYGFNGNVTGDDTGDIGGLIGANVSIGHTLKYVQPDFKTILESPTDKKVGWKVIFNNMVNQNWGPYDRDSWNPVYGNQLFMKTRNGSMKAADNFLDPNKASSLLSSGFSPDFATVITMDRKASKQQTNIDVIYERVRDDYQLHWTSTNWKGTNTKDKWTDRSSERYKIDWEKEEMTNGLSAWSHPQFEK

SEQ ID NO: 89 - protein, 305 aa, Artificial Sequence
  aHL variant
ADSDINIDTGTTNIGSNTTVKTGDLVTYDKENGMGKKVFYSFIDDKNHNKKLLVIRTKGTIAGQYRVYSEEGANKSGLAWPSAFKVQLQLPDNEVAQISDYYPRNSIDTKEYMSTLTYGFNGNVTGDDTGKIGGLIGANVSIGHTLKYVQPDFKTILESPTDKKVGWKVIFNNMVNQNWGPYDRDSWNPVYGNQLFMKTRNGSMKAADNFLDPNKASSLLSSGFSPDFATVITMDRKASKQQTNIDVIYERVRDDYQLHWTSTNWKGTNTKDKWTDRSSERYKIDWEDEEMTNGLSAWSHPQFEK

SEQ ID NO: 90 - protein, 305 aa, Artificial Sequence
  aHL variant
ADSDINIDTGTTNIGSNTTVKTGDLVTYDKENGMGKKVFYSFIDDKNHNKKLLVIRTKGTIAGQYRVYSEEGANKSGLAWPSAFKVQLQLPDNEVAQISDYYPRNSIDTKAYMSTLTYGFNGNVTGDDTGKIGGLIGANVSIGHTLKYVQPDFKTILESPTDKKVGWKVIFNNMVNQNWGPYDRDSWNPVYGNQLFMKTRNGSMKAADNFLDPNKASSLLSSGFSPDFATVITMDRKASKQQTNIDVIYERVRDDYQLHWTSTNWKGTNTKDKWTDRSSERYKIDWEKEEMTNGLSAWSHPQFEK

SEQ ID NO: 91 - protein, 305 aa, Artificial Sequence
  aHL variant
ADSDINIDTGTTNIGSNTTVKTGDLVTYDKENGMGKKVFYSFIDDDNHNKKLLVIRTKGTIAGQYRVYSEEGANKSGLAWPSAFKVQLQLPDNEVAQISDYYPRNSIDTKAYDSTLTYGFDGNVTGDDTGKIGGLIGANVSIGHTLKYVQPDFKTILESPTDKKVGWKVIFNNMVNQNWGPYDRDSWNPVYGNQLFMKTRNGSMKAADNFLDPNKASSLLSSGFSPDFATVITMDRKASKQQTNIDVIYERVRDDYQLHWTSTNWKGTNTKDKWTDRSSERYKIDWEKEEMTNGLSAWSHPQFEK

SEQ ID NO: 92 - protein, 305 aa, Artificial Sequence
  aHL variant
DDSDINIKTGTTDIGSDTTVKTGDLVTYDKENGMLKKVFYSFIDDKNHNKKLLVIRTKGTIAGQYRVYSEEGANKSGLAWPSAFKVQLQLPDNEVAQISDYYPRNSIDTKEYMSTLTYGFNGNVTGDDTGDIDGLIGANVSIGHTLDYVQPDFKTILESPTDKKVGWKVIFNNMVNQNWGPYDRDSWNPVYGNQLFMKTRNGSMKAADNFLDPNKASSLLSSGFSPDFATVITMDRKASKQQTNIDVIYERVRDDYQLHWTSTNWKGTNTKDKWTDRSSERYKIDWEKEEMTNGLSAWSHPQFEK

SEQ ID NO: 93 - protein, 305 aa, Artificial Sequence
  aHL variant
DDSDINIKTGTTDIGSDTTVKTGDLVTYDKENGMLKKVFYSFIDDKNHNKKLLVIRTKGTIAGQYRVYSEEGANKSGLAWPSAFKVQLQLPDNEVAQISDYYPRNSIDTKEYMSTLTYGFNGNVTGDDTGDIKGDIGANVSIGHTLDYVQPDFKTILESPTDKKVGWKVIFNNMVNQNWGPYDRDSWNPVYGNQLFMKTRNGSMKAADNFLDPNKASSLLSSGFSPDFATVITMDRKASKQQTNIDVIYERVRDDYQLHWTSTNWKGTNTKDKWTDRSSERYKIDWEKEEMTNGLSAWSHPQFEK

SEQ ID NO: 94 - protein, 305 aa, Artificial Sequence
  aHL variant
ADSDINIDTGTTDIGSDTTVKTGDLVTYDKENGMLKKVFYSFIDDKDHNKKLLVIRTKGTIAGQYRVYSEEGANKSGLAWPSAFKVQLQLPDNEVAQISDYYPRNSIDTKEYDSDLDYGFDGNVTGDDTGKIGGLIGANVSIGHTLAYVQPDFKTILESPTDKKVGWKVIFNNMVNQNWGPYDRDSWNPVYGNQLFMKTRNGSMKAADNFLDPNKASSLLSSGFSPNFATVITMDRKASKQQTNIDVIYERVRDDYQLHWTSTNWKGTNTKDKWTDRSSERYKIDWEKEEMTNGLSAWSHPQFEK

SEQ ID NO: 95 - protein, 305 aa, Artificial Sequence
  aHL variant
DDSDINIKTGTTDIGSNTTVKTGDLVTYDKENGMLKKVFYSFIDDKNHNKKLLVIRTKGTIAGQYRVYSEEGANKSGLAWPSAFKVQLQLPDNEVAQISDYYPRNSIDTKEYMSTLTYGFNGNVTGGKTGDIGGLIGANVSIGHTLDYVQPDFKTILESPTDKKVGWKVIFNNMVNQNWGPYDRDSWNPVYGNQLFMKTRNGSMKAADNFLDPNKASSLLSSGFSPDFATVITMDRKASKQQTNIDVIYERVRDDYQLHWTSTNWKGTNTKDKWTDRSSERYKIDWEKEEMTNGLSAWSHPQFEK

SEQ ID NO: 96 - protein, 305 aa, Artificial Sequence
  aHL variant
DDSDINIDTGTTDIGSDTTVKTGDLVTYDKENGMLKKVFYSFIDDKNHNKKLLVIRTKGTIAGQYRVYSEEGANKSGLAWPSAFKVQLQLPDNEVAQISDYYPRNSIDTKEYMSTLTYGFDGNVTGDDTGDIGGLIGANVSIGHTLDYVQPDFKTILESPTDKKVGWKVIFNNMVNQNWGPYDRDSWNPVYGNQLFMKTRNGSMKAADNFLDPNKASSLLSSGFSPDFATVITMDRKASKQQTNIDVIYERVRDDYQLHWTSTNWKGTNTKDKWTDRSSERYKIDWEKEEMTNGLSAWSHPQFEK

SEQ ID NO: 97 - protein, 305 aa, Artificial Sequence
  aHL variant
ADSDINIDDGTTNIGSNTTVKTGDLVTYDKENGMGKKVFYSFIDDDNHNKKLLVIRTKGTIAGQYRVYSEEGANKSGLAWPSAFKVQLQLPDNEVAQISDYYPRNSIDTKEYMSTLTYGFNGNVTGDDTGKIGGLIGANVSIGHTLKYVQPDFKTILESPTDKKVGWKVIFNNMVNQNWGPYDRDSWNPVYGNQLFMKTRNGSMKAADNFLDPNKASSLLSSGFSPDFATVITMDRKASKQQTNIDVIYERVRDDYQLHWTSTNWKGTNTKDKWTDRSSERYKIDWEKEEMTNGLSAWSHPQFEK

SEQ ID NO: 98 - protein, 305 aa, Artificial Sequence
  aHL variant
ADSDINIDDGTTNIGSNTTVKTGDLVTYDKENGMGKKVFYSFIDDKDHNKKLLVIRTKGTIAGQYRVYSEEGANKSGLAWPSAFKVQLQLPDNEVAQISDYYPRNSIDTKEYMSTLTYGFNGNVTGDDTGKIGGLIGANVSIGHTLKYVQPDFKTILESPTDKKVGWKVIFNNMVNQNWGPYDRDSWNPVYGNQLFMKTRNGSMKAADNFLDPNKASSLLSSGFSPDFATVITMDRKASKQQTNIDVIYERVRDDYQLHWTSTNWKGTNTKDKWTDRSSERYKIDWEKEEMTNGLSAWSHPQFEK

SEQ ID NO: 99 - protein, 305 aa, Artificial Sequence
  aHL variant
ADSDINIDDGTTNIGSNTTVKTGDLVTYDKENGMGKKVFYSFIDDDNHNKKLLVIRTKGTIAGQYRVYSEEGANKSGLAWPSAFKVQLQLPDNEVAQISDYYPRNSIDTKEYMSTLTYGFDGNVTGDDTGKIGGLIGANVSIGHTLKYVQPDFKTILESPTDKKVGWKVIFNNMVNQNWGPYDRDSWNPVYGNQLFMKTRNGSMKAADNFLDPNKASSLLSSGFSPDFATVITMDRKASKQQTNIDVIYERVRDDYQLHWTSTNWKGTNTKDKWTDRSSERYKIDWEKEEMTNGLSAWSHPQFEK

SEQ ID NO: 100 - protein, 305 aa, Artificial Sequence
  aHL variant
ADSDINIKTGTTDIGSNDTVKTGDLVTYDKENGMLKKVFYSFIDDKNHNKKLLVIRTKGTIAGQYRVYSEEGANKSGLAWPSAFKVQLQLPDNEVAQISDYYPRNSIDTKEYMSTLTYGFNGNVTGDDTGDIGGLIGANVSIGHTLDYVQPDFKTILESPTDKKVGWKVIFNNMVNQNWGPYDRDSWNPVYGNQLFMKTRNGSMKAADNFLDPNKASSLLSSGFSPDFATVITMDRKASKQQTNIDVIYERVRDDYQLHWTSTNWKGTNTKDKWTDRSSERYKIDWEKEEMTNGLSAWSHPQFEK

SEQ ID NO: 101 - protein, 305 aa, Artificial Sequence
  aHL variant
ADSDININTGTTDIGSNTTVKTGDLVTYDKENGMLKKVFYSFIDDKNHNKKLLVIRTKGTIAGQYRVYSEEGANKSGLAWPSAFKVQLQLPDNEVAQISDYYPRNSIDTKAYDSDLDYGFNGNVTGDDTGKIGGLIGANVSIGHTLAYVQPDFKTILESPTDKKVGWKVIFNNMVNQNWGPYDRDSWNPVYGNQLFMKTRNGSMKAADNFLDPNKASSLLSSGFSPDFATVITMDRKASKQQTNIDVIYERVRDDYQLHWTSTNWKGTNTKDKWTDRSSERYKIDWEKEEMTNGLSAWSHPQFEK

SEQ ID NO: 102 - protein, 45 aa, Artificial Sequence
  Peptide tag construct
  MISC_FEATURE (45)..(45): Carboxy terminus optionally may be converted to amide
KKKPPKKPPKKPPKKPPKKPPKKPPKKPPKKPPKKPPKKPPKKKK

SEQ ID NO: 103 - protein, 46 aa, Artificial Sequence
  Peptide tag construct
  MISC_FEATURE (46)..(46): Carboxy terminus optionally may be converted to amide
KKKPKPKPKPKPKPKPKPKPKPKPKPKPKPKPKPKPKPKPKPKKKK

SEQ ID NO: 104 - protein, 46 aa, Artificial Sequence
  Peptide tag construct
  MISC_FEATURE (1)..(1): N-terminal peptide linkages formed by this amino acid occur via the side chain amine (i.e. epsilon-linked lysine when peptide linkages occur at the N-terminus)
  MISC_FEATURE (46)..(46): Carboxy terminus optionally may be converted to amide
KKKKPPKKPPKKPPKKPPKKPPKKPPKKPPKKPPKKPPKKPPKKKK

SEQ ID NO: 105 - protein, 47 aa, Artificial Sequence
  Peptide tag construct
  MISC_FEATURE (1)..(1): N-terminal peptide linkages formed by this amino acid occur via the side chain amine (i.e. epsilon-linked lysine when peptide linkages occur at the N-terminus)
  MISC_FEATURE (47)..(47): Carboxy terminus optionally may be converted to amide
KKKKPKPKPKPKPKPKPKPKPKPKPKPKPKPKPKPKPKPKPKPKKKK

SEQ ID NO: 106 - protein, 44 aa, Artificial Sequence
  Peptide tag construct
  misc_feature (1)..(1): N-terminal peptide linkages formed by this amino acid occur via the side chain amine (i.e. epsilon-linked lysine when peptide linkages occur at the N-terminus)
  misc_feature (44)..(44): Carboxy terminus optionally may be converted to amide
KRRRPPRRPPRRPPRRPPRRPPRRPPRRPPRRPPRRPPRRPPRR

SEQ ID NO: 107 - protein, 56 aa, Artificial Sequence
  Peptide tag construct
  misc_feature (1)..(1): N-terminal peptide linkages formed by this amino acid occur via the side chain amine (i.e. epsilon-linked lysine when peptide linkages occur at the N-terminus)
  misc_feature (56)..(56): Carboxy terminus optionally may be converted to amide
KRRRPPPRRPPPRRPPPRRPPPRRPPPRRPPPRRPPPRRPPPRRPPPRRPPPRRRR

SEQ ID NO: 108 - protein, 45 aa, Artificial Sequence
  Peptide tag construct
  MISC_FEATURE (1)..(1): N-terminal peptide linkages formed by this amino acid occur via the side chain amine (i.e. epsilon-linked lysine when peptide linkages occur at the N-terminus)
  MISC_FEATURE (2)..(3): G is Aminoethylglycine
  MISC_FEATURE (6)..(7): G is Aminoethylglycine
  MISC_FEATURE (10)..(11): G is Aminoethylglycine
  MISC_FEATURE (14)..(15): G is Aminoethylglycine
  MISC_FEATURE (18)..(19): G is Aminoethylglycine
  MISC_FEATURE (22)..(23): G is Aminoethylglycine
  MISC_FEATURE (26)..(27): G is Aminoethylglycine
  MISC_FEATURE (30)..(31): G is Aminoethylglycine
  MISC_FEATURE (34)..(35): G is Aminoethylglycine
  MISC_FEATURE (38)..(39): G is Aminoethylglycine
  MISC_FEATURE (45)..(45): Carboxy terminus optionally may be converted to amide
KGGPPGGPPGGPPGGPPGGPPGGPPGGPPGGPPGGPPGGPPKKKK

SEQ ID NO: 109 - protein, 35 aa, Artificial Sequence
  Peptide tag construct
  MISC_FEATURE (1)..(1): N-terminal peptide linkages formed by this amino acid occur via the side chain amine (i.e. epsilon-linked lysine when peptide linkages occur at the N-terminus)
  MISC_FEATURE (2)..(2): G is aminoethylglycine
  MISC_FEATURE (5)..(5): G is aminoethylglycine
  MISC_FEATURE (8)..(8): G is aminoethylglycine
  MISC_FEATURE (11)..(11): G is aminoethylglycine
  MISC_FEATURE (14)..(14): G is aminoethylglycine
  MISC_FEATURE (17)..(17): G is aminoethylglycine
  MISC_FEATURE (20)..(20): G is aminoethylglycine
  MISC_FEATURE (23)..(23): G is aminoethylglycine
  MISC_FEATURE (26)..(26): G is aminoethylglycine
  MISC_FEATURE (29)..(29): G is aminoethylglycine
  misc_feature (35)..(35): Carboxy terminus optionally may be converted to amide
KGPPGPPGPPGPPGPPGPPGPPGPPGPPGPPKKKK

SEQ ID NO: 110 - protein, 36 aa, Artificial Sequence
  Peptide tag construct
  misc_feature (1)..(1): N-terminal peptide linkages formed by this amino acid occur via the side chain amine (i.e. epsilon-linked lysine when peptide linkages occur at the N-terminus)
  misc_feature (36)..(36): Carboxy terminus optionally may be converted to amide
KKKKPKKPKKPKKPKKPKKPKKPKKPKKPKKPKKKK

SEQ ID NO: 111 - protein, 56 aa, Artificial Sequence
  Peptide tag construct
  misc_feature (1)..(1): N-terminal peptide linkages formed by this amino acid occur via the side chain amine (i.e. epsilon-linked lysine when peptide linkages occur at the N-terminus)
  misc_feature (56)..(56): Carboxy terminus optionally may be converted to amide
KKKKPPPKKPPPKKPPPKKPPPKKPPPKKPPPKKPPPKKPPPKKPPPKKPPPKKKK

SEQ ID NO: 112 - protein, 35 aa, Artificial Sequence
  Peptide tag construct
  MISC_FEATURE (1)..(1): N-terminal peptide linkages formed by this amino acid occur via the side chain amine (i.e. epsilon-linked lysine when peptide linkages occur at the N-terminus)
  MISC_FEATURE (2)..(3): Epsilon-linked lysine
  MISC_FEATURE (5)..(6): Epsilon-linked lysine
  MISC_FEATURE (8)..(9): Epsilon-linked lysine
  MISC_FEATURE (11)..(12): Epsilon-linked lysine
  MISC_FEATURE (14)..(15): Epsilon-linked lysine
  MISC_FEATURE (17)..(18): Epsilon-linked lysine
  MISC_FEATURE (20)..(21): Epsilon-linked lysine
  MISC_FEATURE (23)..(24): Epsilon-linked lysine
  MISC_FEATURE (26)..(27): Epsilon-linked lysine
  MISC_FEATURE (29)..(30): Epsilon-linked lysine
  misc_feature (35)..(35): Carboxy terminus optionally may be converted to amide
KKKPKKPKKPKKPKKPKKPKKPKKPKKPKKPKKKK

SEQ ID NO: 113 - protein, 44 aa, Artificial Sequence
  Peptide tag construct
  MISC_FEATURE (1)..(1): N-terminal peptide linkages formed by this amino acid occur via the side chain amine (i.e. epsilon-linked lysine when peptide linkages occur at the N-terminus)
  MISC_FEATURE (2)..(2): Epsilon-linked lysine
  MISC_FEATURE (5)..(5): Epsilon-linked lysine
  MISC_FEATURE (8)..(8): Epsilon-linked lysine
  MISC_FEATURE (11)..(11): Epsilon-linked lysine
  MISC_FEATURE (14)..(14): Epsilon-linked lysine
  MISC_FEATURE (17)..(17): Epsilon-linked lysine
  MISC_FEATURE (20)..(20): Epsilon-linked lysine
  MISC_FEATURE (23)..(23): Epsilon-linked lysine
  MISC_FEATURE (26)..(26): Epsilon-linked lysine
  MISC_FEATURE (29)..(29): Epsilon-linked lysine
  misc_feature (44)..(44): Carboxy terminus optionally may be converted to amide
KKPPKKPPKKPPKKPPKKPPKKPPKKPPKKPPKKPPKKPPKKKK

SEQ ID NO: 114 - protein, 35 aa, Artificial Sequence
  Peptide tag construct
  MISC_FEATURE (1)..(1): N-terminal peptide linkages formed by this amino acid occur via the side chain amine (i.e. epsilon-linked lysine when peptide linkages occur at the N-terminus)
  MISC_FEATURE (2)..(2): Epsilon-linked lysine
  MISC_FEATURE (5)..(5): Epsilon-linked lysine
  MISC_FEATURE (8)..(8): Epsilon-linked lysine
  MISC_FEATURE (11)..(11): Epsilon-linked lysine
  MISC_FEATURE (14)..(14): Epsilon-linked lysine
  MISC_FEATURE (17)..(17): Epsilon-linked lysine
  MISC_FEATURE (20)..(20): Epsilon-linked lysine
  MISC_FEATURE (23)..(23): Epsilon-linked lysine
  MISC_FEATURE (26)..(26): Epsilon-linked lysine
  MISC_FEATURE (29)..(29): Epsilon-linked lysine
  misc_feature (35)..(35): Carboxy terminus optionally may be converted to amide
KKPPKPPKPPKPPKPPKPPKPPKPPKPPKPPKKKK

SEQ ID NO: 115 - protein, 44 aa, Artificial Sequence
  Peptide tag construct
  MISC_FEATURE (1)..(1): N-terminal peptide linkages formed by this amino acid occur via the side chain amine (i.e. epsilon-linked lysine when peptide linkages occur at the N-terminus)
  MISC_FEATURE (2)..(2): Epsilon-linked lysine
  MISC_FEATURE (3)..(3): X is 4-Benzyloxyproline
  MISC_FEATURE (5)..(6): Epsilon-linked lysine
  MISC_FEATURE (7)..(7): X is 4-Benzyloxyproline
  MISC_FEATURE (9)..(10): Epsilon-linked lysine
  MISC_FEATURE (11)..(11): X is 4-Benzyloxyproline
  MISC_FEATURE (13)..(14): Epsilon-linked lysine
  MISC_FEATURE (15)..(15): X is 4-Benzyloxyproline
  MISC_FEATURE (17)..(18): Epsilon-linked lysine
  MISC_FEATURE (19)..(19): X is 4-Benzyloxyproline
  MISC_FEATURE (21)..(22): Epsilon-linked lysine
  MISC_FEATURE (23)..(23): X is 4-Benzyloxyproline
  MISC_FEATURE (25)..(26): Epsilon-linked lysine
  MISC_FEATURE (27)..(27): X is 4-Benzyloxyproline
  MISC_FEATURE (29)..(30): Epsilon-linked lysine
  MISC_FEATURE (31)..(31): X is 4-Benzyloxyproline
  MISC_FEATURE (33)..(34): Epsilon-linked lysine
  MISC_FEATURE (35)..(35): X is 4-Benzyloxyproline
  MISC_FEATURE (37)..(38): Epsilon-linked lysine
  MISC_FEATURE (39)..(39): X is 4-Benzyloxyproline
  MISC_FEATURE (44)..(44): Carboxy terminus optionally may be converted to amide
KKXPKKXPKKXPKKXPKKXPKKXPKKXPKKXPKKXPKKXPKKKK

SEQ ID NO: 116 - protein, 45 aa, Artificial Sequence
  Peptide tag construct
  MISC_FEATURE (1)..(1): N-terminal peptide linkages formed by this amino acid occur via the side chain amine (i.e. epsilon-linked lysine when peptide linkages occur at the N-terminus)
  misc_feature (45)..(45): Carboxy terminus optionally may be converted to amide
KKGPPKGPPKGPPKGPPKGPPKGPPKGPPKGPPKGPPKGPPKKKK

SEQ ID NO: 117 - protein, 20 aa, Artificial Sequence
  Peptide tag construct
  MISC_FEATURE (1)..(1): N-terminal peptide linkages formed by this amino acid occur via the side chain amine (i.e. epsilon-linked lysine when peptide linkages occur at the N-terminus)
  MISC_FEATURE (2)..(2): Epsilon-linked lysine
  MISC_FEATURE (5)..(5): Epsilon-linked lysine
  MISC_FEATURE (8)..(8): Epsilon-linked lysine
  MISC_FEATURE (11)..(11): Epsilon-linked lysine
  MISC_FEATURE (14)..(14): Epsilon-linked lysine
  MISC_FEATURE (20)..(20): Carboxy terminus optionally may be converted to amide
KKPPKPPKPPKPPKPPKKKK

SEQ ID NO: 118 - protein, 20 aa, Artificial Sequence
  Peptide tag construct
  MISC_FEATURE (1)..(1): N-terminal peptide linkages formed by this amino acid occur via the side chain amine (i.e. epsilon-linked lysine when peptide linkages occur at the N-terminus)
  MISC_FEATURE (2)..(2): Epsilon-linked lysine
  MISC_FEATURE (5)..(6): Epsilon-linked lysine
  MISC_FEATURE (9)..(10): Epsilon-linked lysine
  MISC_FEATURE (13)..(14): Epsilon-linked lysine
  misc_feature (20)..(20): Carboxy terminus optionally may be converted to amide
KKPPKKPPKKPPKKPPKKKK

SEQ ID NO: 119 - protein, 32 aa, Artificial Sequence
  Peptide tag construct
  MISC_FEATURE (1)..(1): N-terminal peptide linkages formed by this amino acid occur via the side chain amine (i.e. epsilon-linked lysine when peptide linkages occur at the N-terminus)
  MISC_FEATURE (2)..(2): Epsilon-linked lysine
  MISC_FEATURE (5)..(6): Epsilon-linked lysine
  MISC_FEATURE (9)..(10): Epsilon-linked lysine
  MISC_FEATURE (13)..(14): Epsilon-linked lysine
  MISC_FEATURE (17)..(18): Epsilon-linked lysine
  MISC_FEATURE (21)..(22): Epsilon-linked lysine
  MISC_FEATURE (25)..(26): Epsilon-linked lysine
  misc_feature (32)..(32): Carboxy terminus optionally may be converted to amide
KKPPKKPPKKPPKKPPKKPPKKPPKKPPKKKK

SEQ ID NO: 120 - protein, 21 aa, Artificial Sequence
  Peptide tag construct
  misc_feature (1)..(1): N-terminal peptide linkages formed by this amino acid occur via the side chain amine (i.e. epsilon-linked lysine when peptide linkages occur at the N-terminus)
  misc_feature (21)..(21): Carboxy terminus optionally may be converted to amide
KKKPPKKPPKKPPKKPPKKKK

SEQ ID NO: 121 - protein, 33 aa, Artificial Sequence
  Peptide tag construct
  misc_feature (1)..(1): N-terminal peptide linkages formed by this amino acid occur via the side chain amine (i.e. epsilon-linked lysine when peptide linkages occur at the N-terminus)
  misc_feature (33)..(33): Carboxy terminus optionally may be converted to amide
KKKPPKKPPKKPPKKPPKKPPKKPPKKPPKKKK

SEQ ID NO: 122 - protein, 33 aa, Artificial Sequence
  Peptide tag construct
  misc_feature (1)..(1): N-terminal peptide linkages formed by this amino acid occur via the side chain amine (i.e. epsilon-linked lysine when peptide linkages occur at the N-terminus)
  misc_feature (33)..(33): Carboxy terminus optionally may be converted to amide
KKAPPKAPPKAPPKAPPKAPPKAPPKAPPKKKK

SEQ ID NO: 123 - protein, 33 aa, Artificial Sequence
  Peptide tag construct
  misc_feature (1)..(1): N-terminal peptide linkages formed by this amino acid occur via the side chain amine (i.e. epsilon-linked lysine when peptide linkages occur at the N-terminus)
  misc_feature (33)..(33): Carboxy terminus optionally may be converted to amide
KKFPPKFPPKFPPKFPPKFPPKFPPKFPPKKKK

SEQ ID NO: 124 - protein, 33 aa, Artificial Sequence
  Peptide tag construct
  misc_feature (1)..(1): N-terminal peptide linkages formed by this amino acid occur via the side chain amine (i.e. epsilon-linked lysine when peptide linkages occur at the N-terminus)
  misc_feature (33)..(33): Carboxy terminus optionally may be converted to amide
KKHPPKHPPKHPPKHPPKHPPKHPPKHPPKKKK

SEQ ID NO: 125 - protein, 33 aa, Artificial Sequence
  Peptide tag construct
  misc_feature (1)..(1): N-terminal peptide linkages formed by this amino acid occur via the side chain amine (i.e. epsilon-linked lysine when peptide linkages occur at the N-terminus)
  misc_feature (33)..(33): Carboxy terminus optionally may be converted to amide
KKLPPKLPPKLPPKLPPKLPPKLPPKLPPKKKK

SEQ ID NO: 126 - protein, 33 aa, Artificial Sequence
  Peptide tag construct
  misc_feature (1)..(1): N-terminal peptide linkages formed by this amino acid occur via the side chain amine (i.e. epsilon-linked lysine when peptide linkages occur at the N-terminus)
  misc_feature (33)..(33): Carboxy terminus optionally may be converted to amide
KKQPPKQPPKQPPKQPPKQPPKQPPKQPPKKKK

SEQ ID NO: 127 - protein, 33 aa, Artificial Sequence
  Peptide tag construct
  misc_feature (1)..(1): N-terminal peptide linkages formed by this amino acid occur via the side chain amine (i.e. epsilon-linked lysine when peptide linkages occur at the N-terminus)
  misc_feature (33)..(33): Carboxy terminus optionally may be converted to amide
KKSPPKSPPKSPPKSPPKSPPKSPPKSPPKKKK

SEQ ID NO: 128 - protein, 33 aa, Artificial Sequence
  Peptide tag construct
  misc_feature (1)..(1): X is propargylglycine
  misc_feature (33)..(33): Carboxy terminus optionally may be converted to amide
XKKPPKKPPKKPPKKPPKKPPKKPPKKPPKKKK

SEQ ID NO: 129 - protein, 33 aa, Artificial Sequence; identical to SEQ ID NO: 128
  Peptide tag construct
  misc_feature (1)..(1): X is Propargylglycine
  misc_feature (2)..(3): Epsilon-linked lysine
  misc_feature (6)..(7): Epsilon-linked lysine
  misc_feature (10)..(11): Epsilon-linked lysine
  misc_feature (14)..(15): Epsilon-linked lysine
  misc_feature (18)..(19): Epsilon-linked lysine
  misc_feature (22)..(23): Epsilon-linked lysine
  misc_feature (26)..(27): Epsilon-linked lysine
  misc_feature (33)..(33): Carboxy terminus optionally may be converted to amide

SEQ ID NO: 130 - protein, 33 aa, Artificial Sequence; identical to SEQ ID NO: 128
  Peptide tag construct
  misc_feature (1)..(1): X is Pyrrolyl alanine (PyrAla)
  misc_feature (33)..(33): Carboxy terminus optionally may be converted to amide

SEQ ID NO: 131 - protein, 45 aa, Artificial Sequence; identical to SEQ ID NO: 102
  Peptide tag construct
  misc_feature (1)..(1): N-terminal peptide linkages formed by this amino acid occur via the side chain amine (i.e. epsilon-linked lysine when peptide linkages occur at the N-terminus)
  misc_feature (45)..(45): Carboxy terminus optionally may be converted to amide

SEQ ID NO: 132 - protein, 57 aa, Artificial Sequence
  Peptide tag construct
  misc_feature (1)..(1): N-terminal peptide linkages formed by this amino acid occur via the side chain amine (i.e. epsilon-linked lysine when peptide linkages occur at the N-terminus)
  misc_feature (57)..(57): Carboxy terminus optionally may be converted to amide
KKKPPKKPPKKPPKKPPKKPPKKPPKKPPKKPPKKPPKKPPKKPPKKPPKKPPKKKK

SEQ ID NO: 133 - protein, 69 aa, Artificial Sequence
  Peptide tag construct
  misc_feature (1)..(1): N-terminal peptide linkages formed by this amino acid occur via the side chain amine (i.e. epsilon-linked lysine when peptide linkages occur at the N-terminus)
  misc_feature (69)..(69): Carboxy terminus optionally may be converted to amide
KKKPPKKPPKKPPKKPPKKPPKKPPKKPPKKPPKKPPKKPPKKPPKKPPKKPPKKPPKKPPKKPPKKKK

SEQ ID NO: 134 - protein, 49 aa, Artificial Sequence
  Peptide tag construct
  misc_feature (1)..(1): N-terminal peptide linkages formed by this amino acid occur via the side chain amine (i.e. epsilon-linked lysine when peptide linkages occur at the N-terminus)
  misc_feature (49)..(49): Carboxy terminus optionally may be converted to amide
KKKPPKKPPKKPPKKPPKKPPKKPPKKPPKKPPKKPPKKPPKKKKKKKK

SEQ ID NO: 135 - protein, 45 aa, Artificial Sequence
  Peptide tag construct
  misc_feature (1)..(1): N-terminal peptide linkages formed by this amino acid occur via the side chain amine (i.e. epsilon-linked lysine when peptide linkages occur at the N-terminus)
  misc_feature (42)..(45): X is 2,3-Diaminopropionic Acid
  misc_feature (45)..(45): Carboxy terminus optionally may be converted to amide
KKKPPKKPPKKPPKKPPKKPPKKPPKKPPKKPPKKPPKKPPXXXX

SEQ ID NO: 136 - protein, 45 aa, Artificial Sequence
  Peptide tag construct
  misc_feature (1)..(1): N-terminal peptide linkages formed by this amino acid occur via the side chain amine (i.e. epsilon-linked lysine when peptide linkages occur at the N-terminus)
  misc_feature (45)..(45): Carboxy terminus optionally may be converted to amide
KKKPPKKPPKKPPKKPPKKPPKKPPKKPPKKPPKKPPKKPPRRRR

SEQ ID NO: 137 - protein, 49 aa, Artificial Sequence
  Peptide tag construct
  misc_feature (1)..(1): N-terminal peptide linkages formed by this amino acid occur via the side chain amine (i.e. epsilon-linked lysine when peptide linkages occur at the N-terminus)
  misc_feature (49)..(49): Carboxy terminus optionally may be converted to amide
KKKPPKKPPKKPPKKPPKKPPKKPPKKPPKKPPKKPPKKPPRRRRRRRR

SEQ ID NO: 138 - protein, 45 aa, Artificial Sequence; identical to SEQ ID NO: 135
  Peptide tag construct
  misc_feature (1)..(1): N-terminal peptide linkages formed by this amino acid occur via the side chain amine (i.e. epsilon-linked lysine when peptide linkages occur at the N-terminus)
  misc_feature (42)..(45): X is Dap-aminoethyl
  misc_feature (45)..(45): Carboxy terminus optionally may be converted to amide

SEQ ID NO: 139 - protein, 35 aa, Artificial Sequence
  Peptide tag construct
  misc_feature (1)..(1): N-terminal peptide linkages formed by this amino acid occur via the side chain amine (i.e. epsilon-linked lysine when peptide linkages occur at the N-terminus)
  misc_feature (2)..(2): A is beta-alanine
  misc_feature (4)..(4): A is beta-alanine
  misc_feature (6)..(6): A is beta-alanine
  misc_feature (8)..(8): A is beta-alanine
  misc_feature (10)..(10): A is beta-alanine
  misc_feature (12)..(12): A is beta-alanine
  misc_feature (14)..(14): A is beta-alanine
  misc_feature (16)..(16): A is beta-alanine
  misc_feature (18)..(18): A is beta-alanine
  misc_feature (20)..(20): A is beta-alanine
  misc_feature (22)..(22): A is beta-alanine
  misc_feature (24)..(24): A is beta-alanine
  misc_feature (26)..(26): A is beta-alanine
  misc_feature (28)..(28): A is beta-alanine
  misc_feature (30)..(30): A is beta-alanine
  misc_feature (35)..(35): Carboxy terminus optionally may be converted to amide
KAKAKAKAKAKAKAKAKAKAKAKAKAKAKAKKKKK

SEQ ID NO: 140 - protein, 35 aa, Artificial Sequence
  Peptide tag construct
  misc_feature (1)..(1): N-terminal peptide linkages formed by this amino acid occur via the side chain amine (i.e. epsilon-linked lysine when peptide linkages occur at the N-terminus)
  misc_feature (2)..(3): A is beta-alanine
  misc_feature (5)..(6): A is beta-alanine
  misc_feature (8)..(9): A is beta-alanine
  misc_feature (11)..(12): A is beta-alanine
  misc_feature (14)..(15): A is beta-alanine
  misc_feature (17)..(18): A is beta-alanine
  misc_feature (20)..(21): A is beta-alanine
  misc_feature (23)..(24): A is beta-alanine
  misc_feature (26)..(27): A is beta-alanine
  misc_feature (29)..(30): A is beta-alanine
  misc_feature (35)..(35): Carboxy terminus optionally may be converted to amide
KAAKAAKAAKAAKAAKAAKAAKAAKAAKAAKKKKK

SEQ ID NO: 141 - protein, 20 aa, Artificial Sequence
  Peptide tag construct
  misc_feature (1)..(1): N-terminal peptide linkages formed by this amino acid occur via the side chain amine (i.e. epsilon-linked lysine when peptide linkages occur at the N-terminus)
  misc_feature (2)..(16): X is Aminoethyl-piperazineacetic acid
  misc_feature (20)..(20): Carboxy terminus optionally may be converted to amide
KXXXXXXXXXXXXXXXKKKK

SEQ ID NO: 142 - protein, 15 aa, Artificial Sequence
  Peptide tag construct
  misc_feature (1)..(1): N-terminal peptide linkages formed by this amino acid occur via the side chain amine (i.e. epsilon-linked lysine when peptide linkages occur at the N-terminus)
  misc_feature (2)..(11): X is Diethylenetriamine-succinamic acid
  misc_feature (15)..(15): Carboxy terminus optionally may be converted to amide
KXXXXXXXXXXKKKK

SEQ ID NO: 143 - protein, 21 aa, Artificial Sequence
  Peptide tag construct
  misc_feature (1)..(1): N-terminal peptide linkages formed by this amino acid occur via the side chain amine (i.e. epsilon-linked lysine when peptide linkages occur at the N-terminus)
  misc_feature (2)..(2): X is Diethylenetriamine-succinamic acid
  misc_feature (3)..(3): X is 2,3-Diaminopropionic Acid
  misc_feature (4)..(4): X is Diethylenetriamine-succinamic acid
  misc_feature (5)..(5): X is 2,3-Diaminopropionic Acid
  misc_feature (6)..(6): X is Diethylenetriamine-succinamic acid
  misc_feature (7)..(7): X is 2,3-Diaminopropionic Acid
  misc_feature (8)..(8): X is Diethylenetriamine-succinamic acid
  misc_feature (9)..(9): X is 2,3-Diaminopropionic Acid
  misc_feature (10)..(10): X is Diethylenetriamine-succinamic acid
  misc_feature (11)..(11): X is 2,3-Diaminopropionic Acid
  misc_feature (12)..(12): X is Diethylenetriamine-succinamic acid
  misc_feature (13)..(13): X is 2,3-Diaminopropionic Acid
  misc_feature (14)..(14): X is Diethylenetriamine-succinamic acid
  misc_feature (15)..(15): X is 2,3-Diaminopropionic Acid
  misc_feature (16)..(16): X is Diethylenetriamine-succinamic acid
  misc_feature (17)..(17): X is 2,3-Diaminopropionic Acid
  misc_feature (21)..(21): Carboxy terminus optionally may be converted to amide
KXXXXXXXXXXXXXXXXKKKK

SEQ ID NO: 144 - protein, 13 aa, Artificial Sequence
  Peptide tag construct
  misc_feature (1)..(1): N-terminal peptide linkages formed by this amino acid occur via the side chain amine (i.e. epsilon-linked lysine when peptide linkages occur at the N-terminus)
  misc_feature (2)..(9): x is Triethylenetriamine-succinamic acid
  misc_feature (13)..(13): Carboxy terminus optionally may be converted to amide
KXXXXXXXXKKKK

SEQ ID NO: 145 - protein, 45 aa, Artificial Sequence
  Peptide tag construct
  misc_feature (1)..(1): N-terminal peptide linkages formed by this amino acid occur via the side chain amine (i.e. epsilon-linked lysine when peptide linkages occur at the N-terminus)
  misc_feature (45)..(45): Carboxy terminus optionally may be converted to amide
KKAAAKAAAKAAAKAAAKAAAKAAAKAAAKAAAKAAAKAAAKKKK

SEQ ID NO: 146 - protein, 45 aa, Artificial Sequence
  Peptide tag construct
  misc_feature (1)..(1): N-terminal peptide linkages formed by this amino acid occur via the side chain amine (i.e. epsilon-linked lysine when peptide linkages occur at the N-terminus)
  misc_feature (45)..(45): Carboxy terminus optionally may be converted to amide
KKGKGKGKGKGKGKGKGKGKGKGKGKGKGKGKGKGKGKGKGKKKK

SEQ ID NO: 147 - protein, 45 aa, Artificial Sequence
  Peptide tag construct
  misc_feature (1)..(1): N-terminal peptide linkages formed by this amino acid occur via the side chain amine (i.e. epsilon-linked lysine when peptide linkages occur at the N-terminus)
  misc_feature (45)..(45): Carboxy terminus optionally may be converted to amide
KKKGGKKGGKKGGKKGGKKGGKKGGKKGGKKGGKKGGKKGGKKKK

SEQ ID NO: 148 - protein, 45 aa, Artificial Sequence
  Peptide tag construct
  misc_feature (1)..(1): N-terminal peptide linkages formed by this amino acid occur via the side chain amine (i.e. epsilon-linked lysine when peptide linkages occur at the N-terminus)
  misc_feature (45)..(45): Carboxy terminus optionally may be converted to amide
KKKGPKKGPKKGPKKGPKKGPKKGPKKGPKKGPKKGPKKGPKKKK

SEQ ID NO: 149 - protein, 45 aa, Artificial Sequence
  Peptide tag construct
  misc_feature (1)..(1): N-terminal peptide linkages formed by this amino acid occur via the side chain amine (i.e. epsilon-linked lysine when peptide linkages occur at the N-terminus)
  misc_feature (2)..(3): X is 4-aminoproline
  misc_feature (6)..(7): X is 4-aminoproline
  misc_feature (10)..(11): X is 4-aminoproline
  misc_feature (14)..(15): X is 4-aminoproline
  misc_feature (18)..(19): X is 4-aminoproline
  misc_feature (22)..(23): X is 4-aminoproline
  misc_feature (26)..(27): X is 4-aminoproline
  misc_feature (30)..(31): X is 4-aminoproline
  misc_feature (34)..(35): X is 4-aminoproline
  misc_feature (38)..(39): X is 4-aminoproline
  misc_feature (45)..(45): Carboxy terminus optionally may be converted to amide
KXXPPXXPPXXPPXXPPXXPPXXPPXXPPXXPPXXPPXXPPKKKK

SEQ ID NO: 150 - protein, 45 aa, Artificial Sequence
  Peptide tag construct
  misc_feature (1)..(1): N-terminal peptide linkages formed by this amino acid occur via the side chain amine (i.e. epsilon-linked lysine when peptide linkages occur at the N-terminus)
  misc_feature (2)..(2): X is 4-aminoproline
  misc_feature (4)..(4): X is 4-aminoproline
  misc_feature (6)..(6): X is 4-aminoproline
  misc_feature (8)..(8): X is 4-aminoproline
  misc_feature (10)..(10): X is 4-aminoproline
  misc_feature (12)..(12): X is 4-aminoproline
  misc_feature (14)..(14): X is 4-aminoproline
  misc_feature (16)..(16): X is 4-aminoproline
  misc_feature (18)..(18): X is 4-aminoproline
  misc_feature (20)..(20): X is 4-aminoproline
  misc_feature (22)..(22): X is 4-aminoproline
  misc_feature (24)..(24): X is 4-aminoproline
  misc_feature (26)..(26): X is 4-aminoproline
  misc_feature (28)..(28): X is 4-aminoproline
  misc_feature (30)..(30): X is 4-aminoproline
  misc_feature (32)..(32): X is 4-aminoproline
  misc_feature (34)..(34): X is 4-aminoproline
  misc_feature (36)..(36): X is 4-aminoproline
  misc_feature (38)..(38): X is 4-aminoproline
  misc_feature (40)..(40): X is 4-aminoproline
  misc_feature (45)..(45): Carboxy terminus optionally may be converted to amide
KXPXPXPXPXPXPXPXPXPXPXPXPXPXPXPXPXPXPXPXPKKKK

SEQ ID NO: 151 - protein, 45 aa, Artificial Sequence
  Peptide tag construct
  misc_feature (1)..(1): N-terminal peptide linkages formed by this amino acid occur via the side chain amine (i.e. epsilon-linked lysine when peptide linkages occur at the N-terminus)
  misc_feature (2)..(41): X is 4-aminoproline
  misc_feature (45)..(45): Carboxy terminus optionally may be converted to amide
KXXXXXXXXXXXXXXXXXXXXXXXXXXXXXXXXXXXXXXXXKKKK

SEQ ID NO: 152 - protein, 40 aa, Artificial Sequence
  Peptide tag construct
  misc_feature (40)..(40): Carboxy terminus optionally may be converted to amide
KKKKKKKKKKKKKKKKKKKKKKKKKKKKKKKKKKKKKKKK

SEQ ID NO: 153 - protein, 35 aa, Artificial Sequence; identical to SEQ ID NO: 112
  Peptide tag construct
  misc_feature (1)..(1): Epsilon-linked lysine
  misc_feature (35)..(35): Carboxy terminus optionally may be converted to amide

SEQ ID NO: 154 - protein, 55 aa, Artificial Sequence
  Peptide tag construct
  misc_feature (1)..(1): Epsilon-linked lysine
  misc_feature (55)..(55): Carboxy terminus optionally may be converted to amide
KKKPPPKKPPPKKPPPKKPPPKKPPPKKPPPKKPPPKKPPPKKPPPKKPPPKKKK

SEQ ID NO: 155 - protein, 35 aa, Artificial Sequence
  Peptide tag
  MISC_FEATURE (1)..(1): X is 4-nitrophenylalanine (4NPA)
  MISC_FEATURE (2)..(3): Epsilon-linked lysine
  MISC_FEATURE (5)..(6): Epsilon-linked lysine
  MISC_FEATURE (8)..(9): Epsilon-linked lysine
  MISC_FEATURE (11)..(12): Epsilon-linked lysine
  MISC_FEATURE (14)..(15): Epsilon-linked lysine
  MISC_FEATURE (17)..(18): Epsilon-linked lysine
  MISC_FEATURE (20)..(21): Epsilon-linked lysine
  MISC_FEATURE (23)..(24): Epsilon-linked lysine
  MISC_FEATURE (26)..(27): Epsilon-linked lysine
  MISC_FEATURE (29)..(30): Epsilon-linked lysine
  MISC_FEATURE (35)..(35): Carboxy terminus optionally may be converted to amide
XKKPKKPKKPKKPKKPKKPKKPKKPKKPKKPKKKK

SEQ ID NO: 156 - protein, 25 aa, Artificial Sequence
  Peptide tag
  MISC_FEATURE (1)..(1): X is 4-nitrophenylalanine
  MISC_FEATURE (2)..(21): Epsilon-linked lysine
  MISC_FEATURE (25)..(25): Carboxy terminus optionally may be converted to amide
XKKKKKKKKKKKKKKKKKKKKKKKK

SEQ ID NO: 157 - protein, 35 aa, Artificial Sequence
  Peptide tag
  MISC_FEATURE (1)..(1): X is 4-nitrophenylalanine
  MISC_FEATURE (2)..(2): X is Aminoethylglycine
  MISC_FEATURE (5)..(5): X is Aminoethylglycine
  MISC_FEATURE (8)..(8): X is Aminoethylglycine
  MISC_FEATURE (11)..(11): X is Aminoethylglycine
  MISC_FEATURE (14)..(14): X is Aminoethylglycine
  MISC_FEATURE (17)..(17): X is Aminoethylglycine
  MISC_FEATURE (20)..(20): X is Aminoethylglycine
  MISC_FEATURE (23)..(23): X is Aminoethylglycine
  MISC_FEATURE (26)..(26): X is Aminoethylglycine
  MISC_FEATURE (29)..(29): X is Aminoethylglycine
  MISC_FEATURE (35)..(35): Carboxy terminus optionally may be converted to amide
XXPPXPPXPPXPPXPPXPPXPPXPPXPPXPPKKKK

SEQ ID NO: 158 - protein, 4 aa, Artificial Sequence
  Polymer tag
  MISC_FEATURE (1)..(2): x = diaminopropionic acid
XXPP

SEQ ID NO: 159 - protein, 4 aa, Artificial Sequence
  Repeat unit of polymer tag
  MISC_FEATURE (1)..(2): x = epsilon-linked lysine
XXGG

SEQ ID NO: 160 - protein, 5 aa, Artificial Sequence
  Repeat unit for polymer tag
  MISC_FEATURE (2)..(2): X = Lysine-Peg
  MISC_FEATURE (4)..(4): X = Lysine-Peg
GXGXP

SEQ ID NO: 161 - protein, 4 aa, Artificial Sequence
  Repeat unit for polymer tag
  MISC_FEATURE (2)..(3): x = Lysine-Peg4
GXXP

SEQ ID NO: 162 - protein, 4 aa, Artificial Sequence
  Repeat unit for polymer tag
  MISC_FEATURE (1)..(1): x = (Aminoethyl)-glycine
  MISC_FEATURE (2)..(4): x = Peptide Nucleic Acid (Thymine)
XXXX

SEQ ID NO: 163 - protein, 5 aa, Artificial Sequence
  Repeat unit for polymer tag
  MISC_FEATURE (2)..(2): x = Lysine-Peg3
  MISC_FEATURE (4)..(4): x = Lysine-Peg3
GXGXP

SEQ ID NO: 164 - protein, 5 aa, Artificial Sequence
  Repeat unit for polymer tag
  MISC_FEATURE (1)..(1): x = epsilon-linked lysine
XRPPP

SEQ ID NO: 165 - protein, 4 aa, Artificial Sequence
  Repeat unit for polymer tag
KKKP

SEQ ID NO: 166 - protein, 4 aa, Artificial Sequence
  Repeat unit for polymer tag
KPRP

SEQ ID NO: 167 - protein, 4 aa, Artificial Sequence
  Repeat unit for polymer tag
KKRP

SEQ ID NO: 168 - protein, 25 aa, Artificial Sequence
  Polymer tag
  MISC_FEATURE (1)..(1): x = Hexynyl-4-Nitrophenylalanine
  MISC_FEATURE (2)..(21): x = epsilon-linked lysine
  MISC_FEATURE (25)..(25): Carboxy terminus optionally may be converted to amide
XXXXXXXXXXXXXXXXXXXXXKKKK

SEQ ID NO: 169 - protein, 35 aa, Artificial Sequence; identical to SEQ ID NO: 157
  Polymer tag
  MISC_FEATURE (1)..(1): x = hexynyl-4-nitrophenylalanine
  MISC_FEATURE (2)..(2): x = (Aminoethyl)-glycine
  MISC_FEATURE (5)..(5): x = (Aminoethyl)-glycine
  MISC_FEATURE (8)..(8): x = (Aminoethyl)-glycine
  MISC_FEATURE (11)..(11): x = (Aminoethyl)-glycine
  MISC_FEATURE (14)..(14): x = (Aminoethyl)-glycine
  MISC_FEATURE (17)..(17): x = (Aminoethyl)-glycine
  MISC_FEATURE (20)..(20): x = (Aminoethyl)-glycine
  MISC_FEATURE (23)..(23): x = (Aminoethyl)-glycine
  MISC_FEATURE (26)..(26): x = (Aminoethyl)-glycine
  MISC_FEATURE (29)..(29): x = (Aminoethyl)-glycine
  MISC_FEATURE (35)..(35): Carboxy terminus optionally may be converted to amide

SEQ ID NO: 170 - protein, 35 aa, Artificial Sequence
  Polymer tag
  MISC_FEATURE (1)..(1): x = hexynyl-4-nitrophenylalanine
  MISC_FEATURE (2)..(3): x = epsilon-linked lysine
  MISC_FEATURE (5)..(6): x = epsilon-linked lysine
  MISC_FEATURE (8)..(9): x = epsilon-linked lysine
  MISC_FEATURE (11)..(12): x = epsilon-linked lysine
  MISC_FEATURE (14)..(15): x = epsilon-linked lysine
  MISC_FEATURE (17)..(18): x = epsilon-linked lysine
  MISC_FEATURE (20)..(21): x = epsilon-linked lysine
  MISC_FEATURE (23)..(24): x = epsilon-linked lysine
  MISC_FEATURE (26)..(27): x = epsilon-linked lysine
  MISC_FEATURE (29)..(30): x = epsilon-linked lysine
  MISC_FEATURE (35)..(35): Carboxy terminus optionally may be converted to amide
XXXPXXPXXPXXPXXPXXPXXPXXPXXPXXPKKKK

SEQ ID NO: 171 - protein, 45 aa, Artificial Sequence
  Polymer tag
  MISC_FEATURE (1)..(1): x = hexynyl-4-nitrophenylalanine
  MISC_FEATURE (2)..(3): x = (Aminoethyl)-glycine
  MISC_FEATURE (6)..(7): x = (Aminoethyl)-glycine
  MISC_FEATURE (10)..(11): x = (Aminoethyl)-glycine
  MISC_FEATURE (14)..(15): x = (Aminoethyl)-glycine
  MISC_FEATURE (18)..(19): x = (Aminoethyl)-glycine
  MISC_FEATURE (22)..(23): x = (Aminoethyl)-glycine
  MISC_FEATURE (26)..(27): x = (Aminoethyl)-glycine
  MISC_FEATURE (30)..(31): x = (Aminoethyl)-glycine
  MISC_FEATURE (34)..(35): x = (Aminoethyl)-glycine
  MISC_FEATURE (38)..(39): x = (Aminoethyl)-glycine
  MISC_FEATURE (45)..(45): Carboxy terminus optionally may be converted to amide
XXXPPXXPPXXPPXXPPXXPPXXPPXXPPXXPPXXPPXXPPKKKK

SEQ ID NO: 172 - protein, 35 aa, Artificial Sequence; identical to SEQ ID NO: 170
  Polymer tag
  MISC_FEATURE (1)..(1): x = 4-nitrophenylalanine
  MISC_FEATURE (2)..(3): x = (Aminoethyl)-glycine
  MISC_FEATURE (5)..(6): x = (Aminoethyl)-glycine
  MISC_FEATURE (8)..(9): x = (Aminoethyl)-glycine
  MISC_FEATURE (11)..(12): x = (Aminoethyl)-glycine
  MISC_FEATURE (14)..(15): x = (Aminoethyl)-glycine
  MISC_FEATURE (17)..(18): x = (Aminoethyl)-glycine
  MISC_FEATURE (20)..(21): x = (Aminoethyl)-glycine
  MISC_FEATURE (23)..(24): x = (Aminoethyl)-glycine
  MISC_FEATURE (26)..(27): x = (Aminoethyl)-glycine
  MISC_FEATURE (29)..(30): x = (Aminoethyl)-glycine
  MISC_FEATURE (35)..(35): Carboxy terminus optionally may be converted to amide

SEQ ID NO: 173 - protein, 33 aa, Artificial Sequence
  Polymer tag
  MISC_FEATURE (1)..(1): x = Propargylglycine
  MISC_FEATURE (2)..(3): x = epsilon-linked lysine
  MISC_FEATURE (6)..(7): x = epsilon-linked lysine
  MISC_FEATURE (10)..(11): x = epsilon-linked lysine
  MISC_FEATURE (14)..(15): x = epsilon-linked lysine
  MISC_FEATURE (18)..(19): x = epsilon-linked lysine
  MISC_FEATURE (22)..(23): x = epsilon-linked lysine
  MISC_FEATURE (26)..(27): x = epsilon-linked lysine
  MISC_FEATURE (33)..(33): Carboxy terminus optionally may be converted to amide
XXXPPXXPPXXPPXXPPXXPPXXPPXXPPKKKK

SEQ ID NO: 174 - protein, 50 aa, Artificial Sequence
  Polymer tag
  MISC_FEATURE (1)..(1): x = 4-nitrophenylalanine
  MISC_FEATURE (3)..(3): x = 4-Amino-proline
  MISC_FEATURE (6)..(6): x = 4-Amino-proline
  MISC_FEATURE (9)..(9): x = 4-Amino-proline
  MISC_FEATURE (12)..(12): x = 4-Amino-proline
  MISC_FEATURE (15)..(15): x = 4-Amino-proline
  MISC_FEATURE (18)..(18): x = 4-Amino-proline
  MISC_FEATURE (21)..(21): x = 4-Amino-proline
  MISC_FEATURE (24)..(24): x = 4-Amino-proline
  MISC_FEATURE (27)..(27): x = 4-Amino-proline
  MISC_FEATURE (30)..(30): x = 4-Amino-proline
  MISC_FEATURE (33)..(33): x = 4-Amino-proline
  MISC_FEATURE (36)..(36): x = 4-Amino-proline
  MISC_FEATURE (39)..(39): x = 4-Amino-proline
  MISC_FEATURE (42)..(42): x = 4-Amino-proline
  MISC_FEATURE (45)..(45): x = 4-Amino-proline
  MISC_FEATURE (50)..(50): Carboxy terminus optionally may be converted to amide
XGXPGXPGXPGXPGXPGXPGXPGXPGXPGXPGXPGXPGXPGXPGXPKKKK

SEQ ID NO: 175 - protein, 35 aa, Artificial Sequence
  POLYMER TAG
  MISC_FEATURE (1)..(1): x = 4-nitrophenylalanine
  MISC_FEATURE (2)..(3): x = epsilon-linked lysine
  MISC_FEATURE (5)..(6): x = epsilon-linked lysine
  MISC_FEATURE (8)..(9): x = epsilon-linked lysine
  MISC_FEATURE (11)..(12): x = epsilon-linked lysine
  MISC_FEATURE (14)..(15): x = epsilon-linked lysine
  MISC_FEATURE (17)..(18): x = epsilon-linked lysine
  MISC_FEATURE (20)..(21): x = epsilon-linked lysine
  MISC_FEATURE (23)..(24): x = epsilon-linked lysine
  MISC_FEATURE (26)..(27): x = epsilon-linked lysine
  MISC_FEATURE (29)..(30): x = epsilon-linked lysine
  MISC_FEATURE (32)..(35): x = epsilon-linked lysine
  MISC_FEATURE (35)..(35): Carboxy terminus optionally may be converted to amide
XXXPXXPXXPXXPXXPXXPXXPXXPXXPXXPXXXX

SEQ ID NO: 176 - protein, 45 aa, Artificial Sequence
  Polymer tag
  MISC_FEATURE (1)..(1): x = heynyl-4-nitrophenylalanine
  MISC_FEATURE (45)..(45): Carboxy terminus optionally may be converted to amide
XKGKGKGKGKGKGKGKGKGKGKGKGKGKGKGKGKGKGKGKGKKKK

SEQ ID NO: 177 - protein, 35 aa, Artificial Sequence
  Polymer tag
  MISC_FEATURE (1)..(1): x = hexynyl-4-nitrophenylalanine
  MISC_FEATURE (2)..(2): x = epsilon-linked lysine
  MISC_FEATURE (5)..(5): x = epsilon-linked lysine
  MISC_FEATURE (8)..(8): x = epsilon-linked lysine
  MISC_FEATURE (11)..(11): x = epsilon-linked lysine
  MISC_FEATURE (14)..(14): x = epsilon-linked lysine
  MISC_FEATURE (17)..(17): x = epsilon-linked lysine
  MISC_FEATURE (20)..(20): x = epsilon-linked lysine
  MISC_FEATURE (23)..(23): x = epsilon-linked lysine
  MISC_FEATURE (26)..(26): x = epsilon-linked lysine
  MISC_FEATURE (29)..(29): x = epsilon-linked lysine
  MISC_FEATURE (35)..(35): Carboxy terminus optionally may be converted to amide
XXKPXKPXKPXKPXKPXKPXKPXKPXKPXKPKKKK

SEQ ID NO: 178 - protein, 45 aa, Artificial Sequence; identical to SEQ ID NO: 171
  Polymer tag
  MISC_FEATURE (1)..(1): x = hexynyl-4-nitrophenylalanine
  MISC_FEATURE (2)..(3): x = epsilon-linked lysine
  MISC_FEATURE (6)..(7): x = epsilon-linked lysine
  MISC_FEATURE (10)..(11): x = epsilon-linked lysine
  MISC_FEATURE (14)..(15): x = epsilon-linked lysine
  MISC_FEATURE (18)..(19): x = epsilon-linked lysine
  MISC_FEATURE (22)..(23): x = epsilon-linked lysine
  MISC_FEATURE (26)..(27): x = epsilon-linked lysine
  MISC_FEATURE (30)..(31): x = epsilon-linked lysine
  MISC_FEATURE (34)..(35): x = epsilon-linked lysine
  MISC_FEATURE (38)..(39): x = epsilon-linked lysine
  MISC_FEATURE (45)..(45): Carboxy terminus optionally may be converted to amide

SEQ ID NO: 179 - protein, 35 aa, Artificial Sequence
  Polymer tag
  MISC_FEATURE (1)..(1): x = 4-nitrophenylalanine
  MISC_FEATURE (2)..(3): x = epsilon-linked lysine
  MISC_FEATURE (4)..(4): x = Peptide Nucleic Acid (Thymine)
  MISC_FEATURE (5)..(6): x = epsilon-linked lysine
  MISC_FEATURE (7)..(7): x = Peptide Nucleic Acid (Thymine)
  MISC_FEATURE (8)..(9): x = epsilon-linked lysine
  MISC_FEATURE (10)..(10): x = Peptide Nucleic Acid (Thymine)
  MISC_FEATURE (11)..(12): x = epsilon-linked lysine
  MISC_FEATURE (13)..(13): x = Peptide Nucleic Acid (Thymine)
  MISC_FEATURE (14)..(15): x = epsilon-linked lysine
  MISC_FEATURE (16)..(16): x = Peptide Nucleic Acid (Thymine)
  MISC_FEATURE (17)..(18): x = epsilon-linked lysine
  MISC_FEATURE (19)..(19): x = Peptide Nucleic Acid (Thymine)
  MISC_FEATURE (20)..(21): x = epsilon-linked lysine
  MISC_FEATURE (22)..(22): x = Peptide Nucleic Acid (Thymine)
  MISC_FEATURE (23)..(24): x = epsilon-linked lysine
  MISC_FEATURE (25)..(25): x = Peptide Nucleic Acid (Thymine)
  MISC_FEATURE (26)..(27): x = epsilon-linked lysine
  MISC_FEATURE (28)..(28): x = Peptide Nucleic Acid (Thymine)
  MISC_FEATURE (29)..(30): x = epsilon-linked lysine
  MISC_FEATURE (31)..(31): x = Peptide Nucleic Acid (Thymine)
  MISC_FEATURE (35)..(35): Carboxy terminus optionally may be converted to amide
XXXXXXXXXXXXXXXXXXXXXXXXXXXXXXXKKKK

SEQ ID NO: 180 - protein, 57 aa, Artificial Sequence
  Polymer tag
  MISC_FEATURE (1)..(1): x = hexynyl-4-nitrophenylalanine
  MISC_FEATURE (57)..(57): Carboxy terminus optionally may be converted to amide
XKKGGKKGGKKGGKKGGKKGGKKGGKKGGKKGGKKGGKKGGKKGGKKGGKKGGKKKK

SEQ ID NO: 181 - protein, 57 aa, Artificial Sequence
  Polymer tag
  MISC_FEATURE (1)..(1): x = hexynyl=4-nitrophenylalanine
  MISC_FEATURE (2)..(3): x = Gamma-diaminopropionic acid
  MISC_FEATURE (6)..(7): x = Gamma-diaminopropionic acid
  MISC_FEATURE (10)..(11): x = Gamma-diaminopropionic acid
  MISC_FEATURE (14)..(15): x = Gamma-diaminopropionic acid
  MISC_FEATURE (18)..(19): x = Gamma-diaminopropionic acid
  MISC_FEATURE (22)..(23): x = Gamma-diaminopropionic acid
  MISC_FEATURE (26)..(27): x = Gamma-diaminopropionic acid
  MISC_FEATURE (30)..(31): x = Gamma-diaminopropionic acid
  MISC_FEATURE (34)..(35): x = Gamma-diaminopropionic acid
  MISC_FEATURE (38)..(39): x = Gamma-diaminopropionic acid
  MISC_FEATURE (42)..(43): x = Gamma-diaminopropionic acid
  MISC_FEATURE (46)..(47): x = Gamma-diaminopropionic acid
  MISC_FEATURE (50)..(51): x = Gamma-diaminopropionic acid
  MISC_FEATURE (57)..(57): Carboxy terminus optionally may be converted to amide
XXXPPXXPPXXPPXXPPXXPPXXPPXXPPXXPPXXPPXXPPXXPPXXPPXXPPKKKK

SEQ ID NO: 182 - protein, 50 aa, Artificial Sequence
  Polymer tag
  MISC_FEATURE (1)..(1): x = hexynyl-4-nitrophenylalanine
  MISC_FEATURE (2)..(2): x = epsilon-linked lysine
  MISC_FEATURE (3)..(3): x = 4-Aminoproline
  MISC_FEATURE (5)..(5): x = epsilon-linked lysine
  MISC_FEATURE (6)..(6): x = 4-Aminoproline
  MISC_FEATURE (8)..(8): x = epsilon-linked lysine
  MISC_FEATURE (9)..(9): x = 4-Aminoproline
  MISC_FEATURE (11)..(11): x = epsilon-linked lysine
  MISC_FEATURE (12)..(12): x = 4-Aminoproline
  MISC_FEATURE (14)..(14): x = epsilon-linked lysine
  MISC_FEATURE (15)..(15): x = 4-Aminoproline
  MISC_FEATURE (17)..(17): x = epsilon-linked lysine
  MISC_FEATURE (18)..(18): x = 4-Aminoproline
  MISC_FEATURE (20)..(20): x = epsilon-linked lysine
  MISC_FEATURE (21)..(21): x = 4-Aminoproline
  MISC_FEATURE (23)..(23): x = epsilon-linked lysine
  MISC_FEATURE (24)..(24): x = 4-Aminoproline
  MISC_FEATURE (26)..(26): x = epsilon-linked lysine
  MISC_FEATURE (27)..(27): x = 4-Aminoproline
  MISC_FEATURE (29)..(29): x = epsilon-linked lysine
  MISC_FEATURE (30)..(30): x = 4-Aminoproline
  MISC_FEATURE (32)..(32): x = epsilon-linked lysine
  MISC_FEATURE (33)..(33): x = 4-Aminoproline
  MISC_FEATURE (35)..(35): x = epsilon-linked lysine
  MISC_FEATURE (36)..(36): x = 4-Aminoproline
  MISC_FEATURE (38)..(38): x = epsilon-linked lysine
  MISC_FEATURE (39)..(39): x = 4-Aminoproline
  MISC_FEATURE (41)..(41): x = epsilon-linked lysine
  MISC_FEATURE (42)..(42): x = 4-Aminoproline
  MISC_FEATURE (44)..(44): x = epsilon-linked lysine
  MISC_FEATURE (45)..(45): x = 4-Aminoproline
  MISC_FEATURE (50)..(50): Carboxy terminus optionally may be converted to amide
XXXPXXPXXPXXPXXPXXPXXPXXPXXPXXPXXPXXPXXPXXPXXPKKKK

SEQ ID NO: 183 - protein, 20 aa, Artificial Sequence
  Polymer tag
  MISC_FEATURE (1)..(1): x = hexynyl-4-nitrophenylalanine
  MISC_FEATURE (2)..(3): x = epsilon-linked lysine
  MISC_FEATURE (4)..(4): x = Aminohexanoic acid
  MISC_FEATURE (5)..(6): x = epsilon-linked lysine
  MISC_FEATURE (7)..(7): x = Aminohexanoic acid
  MISC_FEATURE (8)..(9): x = epsilon-linked lysine
  MISC_FEATURE (10)..(10): x = Aminohexanoic acid
  MISC_FEATURE (11)..(12): x = epsilon-linked lysine
  MISC_FEATURE (13)..(13): x = Aminohexanoic acid
  MISC_FEATURE (14)..(15): x = epsilon-linked lysine
  MISC_FEATURE (16)..(16): x = Aminohexanoic acid
  MISC_FEATURE (17)..(20): x = epsilon-linked lysine
  MISC_FEATURE (20)..(20): Carboxy terminus optionally may be converted to amide
XXXXXXXXXXXXXXXXXXXX

SEQ ID NO: 184 - protein, 25 aa, Artificial Sequence
  Polymer tag
  MISC_FEATURE (1)..(1): x = hexynyl-4-nitrophenylalanine
  MISC_FEATURE (2)..(3): x = epsilon-linked lysine
  MISC_FEATURE (6)..(7): x = epsilon-linked lysine
  MISC_FEATURE (10)..(11): x = epsilon-linked lysine
  MISC_FEATURE (14)..(15): x = epsilon-linked lysine
  MISC_FEATURE (18)..(19): x = epsilon-linked lysine
  MISC_FEATURE (22)..(25): x = epsilon-linked lysine
  MISC_FEATURE (25)..(25): Carboxy terminus optionally may be converted to amide
XXXGGXXGGXXGGXXGGXXGGXXXX

SEQ ID NO: 185 - protein, 35 aa, Artificial Sequence
  Polymer tag
  MISC_FEATURE (1)..(1): x = hexynyl-4-nitrophenylalanine
  MISC_FEATURE (2)..(3): x = epsilon-lined lysine
  MISC_FEATURE (5)..(6): x = epsilon-lined lysine
  MISC_FEATURE (8)..(9): x = epsilon-lined lysine
  MISC_FEATURE (11)..(12): x = epsilon-lined lysine
  MISC_FEATURE (14)..(15): x = epsilon-lined lysine
  MISC_FEATURE (17)..(18): x = epsilon-lined lysine
  MISC_FEATURE (20)..(21): x = epsilon-lined lysine
  MISC_FEATURE (23)..(24): x = epsilon-lined lysine
  MISC_FEATURE (26)..(27): x = epsilon-lined lysine
  MISC_FEATURE (29)..(30): x = epsilon-lined lysine
  MISC_FEATURE (32)..(35): x = epsilon-lined lysine
  MISC_FEATURE (35)..(35): Carboxy terminus optionally may be converted to amide
XXXGXXGXXGXXGXXGXXGXXGXXGXXGXXGXXXX

SEQ ID NO: 186 - protein, 35 aa, Artificial Sequence
  Polymer tag
  MISC_FEATURE (1)..(1): x = hexynyl-4-nitrophenylalanine
  MISC_FEATURE (2)..(3): x = epsilon-linked lysine
  MISC_FEATURE (5)..(6): x = epsilon-linked lysine
  MISC_FEATURE (8)..(9): x = epsilon-linked lysine
  MISC_FEATURE (11)..(12): x = epsilon-linked lysine
  MISC_FEATURE (14)..(15): x = epsilon-linked lysine
  MISC_FEATURE (17)..(18): x = epsilon-linked lysine
  MISC_FEATURE (20)..(21): x = epsilon-linked lysine
  MISC_FEATURE (23)..(24): x = epsilon-linked lysine
  MISC_FEATURE (26)..(27): x = epsilon-linked lysine
  MISC_FEATURE (29)..(30): x = epsilon-linked lysine
  MISC_FEATURE (32)..(35): x = epsilon-linked lysine
  MISC_FEATURE (35)..(35): Carboxy terminus optionally may be converted to amide
XXXAXXAXXAXXAXXAXXAXXAXXAXXAXXAXXXX

SEQ ID NO: 187 - protein, 35 aa, Artificial Sequence
  Polymer tag
  MISC_FEATURE (1)..(1): x = hexynyl-4-nitrophenylalanine
  MISC_FEATURE (2)..(3): x = epsilon-linked lysine
  MISC_FEATURE (5)..(6): x = epsilon-linked lysine
  MISC_FEATURE (8)..(9): x = epsilon-linked lysine
  MISC_FEATURE (11)..(12): x = epsilon-linked lysine
  MISC_FEATURE (14)..(15): x = epsilon-linked lysine
  MISC_FEATURE (17)..(18): x = epsilon-linked lysine
  MISC_FEATURE (20)..(21): x = epsilon-linked lysine
  MISC_FEATURE (23)..(24): x = epsilon-linked lysine
  MISC_FEATURE (26)..(27): x = epsilon-linked lysine
  MISC_FEATURE (29)..(30): x = epsilon-linked lysine
  MISC_FEATURE (32)..(35): x = epsilon-linked lysine
  MISC_FEATURE (35)..(35): Carboxy terminus optionally may be converted to amide
XXXSXXSXXSXXSXXSXXSXXSXXSXXSXXSXXXX

SEQ ID NO: 188 - protein, 35 aa, Artificial Sequence
  Polymer tag
  MISC_FEATURE (1)..(1): x = hexynyl-4-nitrophenylalanine
  MISC_FEATURE (2)..(3): x = epsilon-linked lysine
  MISC_FEATURE (5)..(6): x = epsilon-linked lysine
  MISC_FEATURE (8)..(9): x = epsilon-linked lysine
  MISC_FEATURE (11)..(12): x = epsilon-linked lysine
  MISC_FEATURE (14)..(15): x = epsilon-linked lysine
  MISC_FEATURE (17)..(18): x = epsilon-linked lysine
  MISC_FEATURE (20)..(21): x = epsilon-linked lysine
  MISC_FEATURE (23)..(24): x = epsilon-linked lysine
  MISC_FEATURE (26)..(27): x = epsilon-linked lysine
  MISC_FEATURE (29)..(30): x = epsilon-linked lysine
  MISC_FEATURE (32)..(35): x = epsilon-linked lysine
  MISC_FEATURE (35)..(35): Carboxy terminus optionally may be converted to amide
XXXFXXFXXFXXFXXFXXFXXFXXFXXFXXFXXXX

SEQ ID NO: 189 - protein, 35 aa, Artificial Sequence
  Polymer tag
  MISC_FEATURE (1)..(1): x = hexynyl-4-nitrophenylalanine
  MISC_FEATURE (2)..(3): x = epsilon-linked lysine
  MISC_FEATURE (4)..(4): x = 4-benzyloxyproline
  MISC_FEATURE (5)..(6): x = epsilon-linked lysine
  MISC_FEATURE (7)..(7): x = 4-benzyloxyproline
  MISC_FEATURE (8)..(9): x = epsilon-linked lysine
  MISC_FEATURE (10)..(10): x = 4-benzyloxyproline
  MISC_FEATURE (11)..(12): x = epsilon-linked lysine
  MISC_FEATURE (13)..(13): x = 4-benzyloxyproline
  MISC_FEATURE (14)..(15): x = epsilon-linked lysine
  MISC_FEATURE (16)..(16): x = 4-benzyloxyproline
  MISC_FEATURE (17)..(18): x = epsilon-linked lysine
  MISC_FEATURE (19)..(19): x = 4-benzyloxyproline
  MISC_FEATURE (20)..(21): x = epsilon-linked lysine
  MISC_FEATURE (22)..(22): x = 4-benzyloxyproline
  MISC_FEATURE (23)..(24): x = epsilon-linked lysine
  MISC_FEATURE (25)..(25): x = 4-benzyloxyproline
  MISC_FEATURE (26)..(27): x = epsilon-linked lysine
  MISC_FEATURE (28)..(28): x = 4-benzyloxyproline
  MISC_FEATURE (29)..(30): x = epsilon-linked lysine
  MISC_FEATURE (31)..(31): x = 4-benzyloxyproline
  MISC_FEATURE (32)..(35): x = epsilon-linked lysine
  MISC_FEATURE (35)..(35): Carboxy terminus optionally may be converted to amide
XXXXXXXXXXXXXXXXXXXXXXXXXXXXXXXXXXX

SEQ ID NO: 190 - protein, 35 aa, Artificial Sequence
  Polymer tag
  MISC_FEATURE (1)..(1): x = hexynyl-4-nitrophenylalanine
  MISC_FEATURE (2)..(3): x = epsilon-linked lysine
  MISC_FEATURE (5)..(6): x = epsilon-linked lysine
  MISC_FEATURE (8)..(9): x = epsilon-linked lysine
  MISC_FEATURE (11)..(12): x = epsilon-linked lysine
  MISC_FEATURE (14)..(15): x = epsilon-linked lysine
  MISC_FEATURE (17)..(18): x = epsilon-linked lysine
  MISC_FEATURE (20)..(21): x = epsilon-linked lysine
  MISC_FEATURE (23)..(24): x = epsilon-linked lysine
  MISC_FEATURE (26)..(27): x = epsilon-linked lysine
  MISC_FEATURE (29)..(30): x = epsilon-linked lysine
  MISC_FEATURE (32)..(35): x = epsilon-linked lysine
  MISC_FEATURE (35)..(35): Carboxy terminus optionally may be converted to amide
XXXQXXQXXQXXQXXQXXQXXQXXQXXQXXQXXXX

SEQ ID NO: 191 - protein, 41 aa, Artificial Sequence
  Polymer tag
  MISC_FEATURE (1)..(1): x = hexynyl-4-nitrophenylalanine
  MISC_FEATURE (2)..(3): x = epsilon-linked lysine
  MISC_FEATURE (5)..(6): x = epsilon-linked lysine
  MISC_FEATURE (8)..(9): x = epsilon-linked lysine
  MISC_FEATURE (11)..(12): x = epsilon-linked lysine
  MISC_FEATURE (14)..(15): x = epsilon-linked lysine
  MISC_FEATURE (17)..(18): x = epsilon-linked lysine
  MISC_FEATURE (20)..(21): x = epsilon-linked lysine
  MISC_FEATURE (23)..(24): x = epsilon-linked lysine
  MISC_FEATURE (26)..(27): x = Peptide Nucleic Acid (Thymine)
  MISC_FEATURE (29)..(30): x = Peptide Nucleic Acid (Thymine)
  MISC_FEATURE (32)..(33): x = Peptide Nucleic Acid (Thymine)
  MISC_FEATURE (35)..(36): x = epsilon-linked lysine
  MISC_FEATURE (38)..(41): x = epsilon-linked lysine
  MISC_FEATURE (41)..(41): Carboxy terminus optionally may be converted to amide
XXXPXXPXXPXXPXXPXXPXXPXXPXXPXXPXXPXXPXXXX

SEQ ID NO: 192 - protein, 41 aa, Artificial Sequence; identical to SEQ ID NO: 191
  Polymer tag
  MISC_FEATURE (1)..(1): x = hexynyl-4-nitrophenylalanine
  MISC_FEATURE (2)..(3): x = epsilon-linked lysine
  MISC_FEATURE (5)..(6): x = epsilon-linked lysine
  MISC_FEATURE (8)..(9): x = epsilon-linked lysine
  MISC_FEATURE (11)..(12): x = epsilon-linked lysine
  MISC_FEATURE (14)..(15): x = epsilon-linked lysine
  MISC_FEATURE (17)..(18): x = epsilon-linked lysine
  MISC_FEATURE (20)..(21): x = peptide nucleic acid (thymine)
  MISC_FEATURE (23)..(24): x = peptide nucleic acid (thymine)
  MISC_FEATURE (26)..(27): x = peptide nucleic acid (thymine)
  MISC_FEATURE (29)..(30): x = epsilon-linked lysine
  MISC_FEATURE (32)..(33): x = epsilon-linked lysine
  MISC_FEATURE (35)..(36): x = epsilon-linked lysine
  MISC_FEATURE (38)..(41): x = epsilon-linked lysine
  MISC_FEATURE (41)..(41): Carboxy terminus optionally may be converted to amide

SEQ ID NO: 193 - protein, 41 aa, Artificial Sequence; identical to SEQ ID NO: 191
  Polymer tag
  MISC_FEATURE (1)..(1): x = hexynyl-4-nitrophenylalanine
  MISC_FEATURE (2)..(3): x = epsilon-linked lysine
  MISC_FEATURE (5)..(6): x = epsilon-linked lysine
  MISC_FEATURE (8)..(9): x = epsilon-linked lysine
  MISC_FEATURE (11)..(12): x = epsilon-linked lysine
  MISC_FEATURE (14)..(15): x = peptide nucleic acid (thymine)
  MISC_FEATURE (17)..(18): x = peptide nucleic acid (thymine)
  MISC_FEATURE (20)..(21): x = peptide nucleic acid (thymine)
  MISC_FEATURE (23)..(24): x = epsilon-linked lysine
  MISC_FEATURE (26)..(27): x = epsilon-linked lysine
  MISC_FEATURE (29)..(30): x = epsilon-linked lysine
  MISC_FEATURE (32)..(33): x = epsilon-linked lysine
  MISC_FEATURE (35)..(36): x = epsilon-linked lysine
  MISC_FEATURE (38)..(41): x = epsilon-linked lysine
  MISC_FEATURE (41)..(41): Carboxy terminus optionally may be converted to amide

SEQ ID NO: 194 - protein, 25 aa, Artificial Sequence
  Polymer tag
  MISC_FEATURE (1)..(1): x = hexynyl-4-nitrophenylalanine
  MISC_FEATURE (2)..(2): x = epsilon-linked lysine
  MISC_FEATURE (3)..(3): x = Oxoaminohexanoic acid
  MISC_FEATURE (4)..(4): x = epsilon-linked lysine
  MISC_FEATURE (5)..(5): x = Oxoaminohexanoic acid
  MISC_FEATURE (6)..(6): x = epsilon-linked lysine
  MISC_FEATURE (7)..(7): x = Oxoaminohexanoic acid
  MISC_FEATURE (8)..(8): x = epsilon-linked lysine
  MISC_FEATURE (9)..(9): x = Oxoaminohexanoic acid
  MISC_FEATURE (10)..(10): x = epsilon-linked lysine
  MISC_FEATURE (11)..(11): x = Oxoaminohexanoic acid
  MISC_FEATURE (12)..(12): x = epsilon-linked lysine
  MISC_FEATURE (13)..(13): x = Oxoaminohexanoic acid
  MISC_FEATURE (14)..(14): x = epsilon-linked lysine
  MISC_FEATURE (15)..(15): x = Oxoaminohexanoic acid
  MISC_FEATURE (16)..(16): x = epsilon-linked lysine
  MISC_FEATURE (17)..(17): x = Oxoaminohexanoic acid
  MISC_FEATURE (18)..(18): x = epsilon-linked lysine
  MISC_FEATURE (19)..(19): x = Oxoaminohexanoic acid
  MISC_FEATURE (20)..(20): x = epsilon-linked lysine
  MISC_FEATURE (21)..(21): x = Oxoaminohexanoic acid
  MISC_FEATURE (22)..(25): x = epsilon-linked lysine
  MISC_FEATURE (25)..(25): Carboxy terminus optionally may be converted to amide
XXXXXXXXXXXXXXXXXXXXXXXXX

SEQ ID NO: 195 - protein, 35 aa, Artificial Sequence; identical to SEQ ID NO: 189
  Polymer tag
  MISC_FEATURE (1)..(1): x = hexynyl-4-nitrophenylalanine
  MISC_FEATURE (2)..(3): x = epsilon-linked lysine
  MISC_FEATURE (4)..(4): x = Oxoaminohexanoic acid
  MISC_FEATURE (5)..(6): x = epsilon-linked lysine
  MISC_FEATURE (7)..(7): x = Oxoaminohexanoic acid
  MISC_FEATURE (8)..(9): x = epsilon-linked lysine
  MISC_FEATURE (10)..(10): x = Oxoaminohexanoic acid
  MISC_FEATURE (11)..(12): x = epsilon-linked lysine
  MISC_FEATURE (13)..(13): x = Oxoaminohexanoic acid
  MISC_FEATURE (14)..(15): x = epsilon-linked lysine
  MISC_FEATURE (16)..(16): x = Oxoaminohexanoic acid
  MISC_FEATURE (17)..(18): x = epsilon-linked lysine
  MISC_FEATURE (19)..(19): x = Oxoaminohexanoic acid
  MISC_FEATURE (20)..(21): x = epsilon-linked lysine
  MISC_FEATURE (22)..(22): x = Oxoaminohexanoic acid
  MISC_FEATURE (23)..(24): x = epsilon-linked lysine
  MISC_FEATURE (25)..(25): x = Oxoaminohexanoic acid
  MISC_FEATURE (26)..(27): x = epsilon-linked lysine
  MISC_FEATURE (28)..(28): x = Oxoaminohexanoic acid
  MISC_FEATURE (29)..(30): x = epsilon-linked lysine
  MISC_FEATURE (31)..(31): x = Oxoaminohexanoic acid
  MISC_FEATURE (32)..(35): x = epsilon-linked lysine
  MISC_FEATURE (35)..(35): Carboxy terminus optionally may be converted to amide

SEQ ID NO: 196 - protein, 9 aa, Artificial Sequence
  Polymer tag
  MISC_FEATURE (1)..(1): x = Propargylglycine
  MISC_FEATURE (2)..(2): x = polyethylene glycol 24mer
  MISC_FEATURE (3)..(3): x = hexynyl
  MISC_FEATURE (4)..(5): x = epsilon-linked lysine
  MISC_FEATURE (9)..(9): Carboxy terminus optionally may be converted to amide
XXXXXKKKK

SEQ ID NO: 197 - protein, 11 aa, Artificial Sequence
  Polymer tag
  MISC_FEATURE (1)..(1): x = Propargylglycine
  MISC_FEATURE (2)..(2): x = polyethylene glycol 24mer
  MISC_FEATURE (3)..(3): x = NHCO
  MISC_FEATURE (4)..(4): x = polyethylene glycol 12mer
  MISC_FEATURE (5)..(5): x = hexynyl
  MISC_FEATURE (6)..(7): x = epsilon-linked lysine
  MISC_FEATURE (11)..(11): Carboxy terminus optionally may be converted to amide
XXXXXXXKKKK

SEQ ID NO: 198 - protein, 11 aa, Artificial Sequence
  Polymer tag
  MISC_FEATURE (1)..(1): x = Propargylglycine
  MISC_FEATURE (2)..(2): x = polyethylene glycol 24mer
  MISC_FEATURE (3)..(3): x = NHCO linkage
  MISC_FEATURE (4)..(4): x = polyethylene glycol 24mer
  MISC_FEATURE (5)..(5): x = hexynyl
  MISC_FEATURE (6)..(7): x = epsilon-linked lysine
  MISC_FEATURE (11)..(11): Carboxy terminus optionally may be converted to amide
XXXXXXXKKKK

SEQ ID NO: 199 - protein, 25 aa, Artificial Sequence
  Polymer tag
  MISC_FEATURE (1)..(1): x = hexynyl-4-nitrophenylalanine
  MISC_FEATURE (2)..(2): x = (Aminoethyl)-glycine
  MISC_FEATURE (3)..(3): x = Oxoaminohexanoic acid
  MISC_FEATURE (4)..(4): x = (Aminoethyl)-glycine
  MISC_FEATURE (5)..(5): x = Oxoaminohexanoic acid
  MISC_FEATURE (6)..(6): x = (Aminoethyl)-glycine
  MISC_FEATURE (7)..(7): x = Oxoaminohexanoic acid
  MISC_FEATURE (8)..(8): x = (Aminoethyl)-glycine
  MISC_FEATURE (9)..(9): x = Oxoaminohexanoic acid
  MISC_FEATURE (10)..(10): x = (Aminoethyl)-glycine
  MISC_FEATURE (11)..(11): x = Oxoaminohexanoic acid
  MISC_FEATURE (12)..(12): x = (Aminoethyl)-glycine
  MISC_FEATURE (13)..(13): x = Oxoaminohexanoic acid
  MISC_FEATURE (14)..(14): x = (Aminoethyl)-glycine
  MISC_FEATURE (15)..(15): x = Oxoaminohexanoic acid
  MISC_FEATURE (16)..(16): x = (Aminoethyl)-glycine
  MISC_FEATURE (17)..(17): x = Oxoaminohexanoic acid
  MISC_FEATURE (18)..(18): x = (Aminoethyl)-glycine
  MISC_FEATURE (19)..(19): x = Oxoaminohexanoic acid
  MISC_FEATURE (20)..(20): x = (Aminoethyl)-glycine
  MISC_FEATURE (21)..(21): x = Oxoaminohexanoic acid
  MISC_FEATURE (22)..(25): x = epsilon-linked lysine
  MISC_FEATURE (25)..(25): Carboxy terminus optionally may be converted to amide
XXXXXXXXXXXXXXXXXXXXXXXXX

SEQ ID NO: 200 - protein, 35 aa, Artificial Sequence; identical to SEQ ID NO: 189
  Polymer tag
  MISC_FEATURE (1)..(1): x = hexynyl-4-nitrophenylalanine
  MISC_FEATURE (2)..(2): x = epsilon-linked lysine
  MISC_FEATURE (3)..(4): x = Oxoaminohexanoic acid
  MISC_FEATURE (5)..(5): x = epsilon-linked lysine
  MISC_FEATURE (6)..(7): x = Oxoaminohexanoic acid
  MISC_FEATURE (8)..(8): x = epsilon-linked lysine
  MISC_FEATURE (9)..(10): x = Oxoaminohexanoic acid
  MISC_FEATURE (11)..(11): x = epsilon-linked lysine
  MISC_FEATURE (12)..(13): x = Oxoaminohexanoic acid
  MISC_FEATURE (14)..(14): x = epsilon-linked lysine
  MISC_FEATURE (15)..(16): x = Oxoaminohexanoic acid
  MISC_FEATURE (17)..(17): x = epsilon-linked lysine
  MISC_FEATURE (18)..(19): x = Oxoaminohexanoic acid
  MISC_FEATURE (20)..(20): x = epsilon-linked lysine
  MISC_FEATURE (21)..(22): x = Oxoaminohexanoic acid
  MISC_FEATURE (23)..(23): x = epsilon-linked lysine
  MISC_FEATURE (24)..(25): x = Oxoaminohexanoic acid
  MISC_FEATURE (26)..(26): x = epsilon-linked lysine
  MISC_FEATURE (27)..(28): x = Oxoaminohexanoic acid
  MISC_FEATURE (29)..(29): x = epsilon-linked lysine
  MISC_FEATURE (30)..(31): x = Oxoaminohexanoic acid
  MISC_FEATURE (32)..(35): x = epsilon-linked lysine
  MISC_FEATURE (35)..(35): Carboxy terminus optionally may be converted to amide

SEQ ID NO: 201 - protein, 15 aa, Artificial Sequence
  Polymer tag
  MISC_FEATURE (1)..(1): x = 4-nitrophenylalanine
  MISC_FEATURE (2)..(2): x = polyethylene glycol 24mer
  MISC_FEATURE (3)..(4): x = peptide nucleic acid (thymine)
  MISC_FEATURE (6)..(7): x = peptide nucleic acid (thymine)
  MISC_FEATURE (9)..(10): x = peptide nucleic acid (thymine)
  MISC_FEATURE (15)..(15): Carboxy terminus optionally may be converted to amide
XXXXPXXPXXPKKKK

SEQ ID NO: 202 - protein, 15 aa, Artificial Sequence
  Polymer tag
  MISC_FEATURE (1)..(1): x = 4-nitrophenylalanine
  MISC_FEATURE (2)..(2): x = polyethylene glycol 24mer
  MISC_FEATURE (3)..(4): x = peptide nucleic acid (thymine)
  MISC_FEATURE (6)..(7): x = peptide nucleic acid (thymine)
  MISC_FEATURE (9)..(10): x = peptide nucleic acid (thymine)
  MISC_FEATURE (15)..(15): Carboxy terminus optionally may be converted to amide
XXXXGXXGXXGKKKK

SEQ ID NO: 203 - protein, 15 aa, Artificial Sequence
  Polymer tag
  MISC_FEATURE (1)..(1): x = 4-nitrophenylalanine
  MISC_FEATURE (2)..(2): x = polyethylene glycol 24mer
  MISC_FEATURE (3)..(4): x = peptide nucleic acid (thymine)
  MISC_FEATURE (6)..(7): x = peptide nucleic acid (thymine)
  MISC_FEATURE (9)..(10): x = peptide nucleic acid (thymine)
  MISC_FEATURE (15)..(15): Carboxy terminus optionally may be converted to amide
XXXXKXXKXXKKKKK

SEQ ID NO: 204 - protein, 8 aa, Artificial Sequence
  Polymer tag
  MISC_FEATURE (1)..(1): x = 4-nitrophenylalanine
  MISC_FEATURE (2)..(2): x = polyethylene glycol 24mer
  MISC_FEATURE (3)..(4): x = epsilon-linked lysine
  MISC_FEATURE (8)..(8): Carboxy terminus optionally may be converted to amide
XXXXKKKK

SEQ ID NO: 205 - protein, 41 aa, Artificial Sequence
  Polymer tag
  MISC_FEATURE (1)..(1): 4-nitrophenylalanine
  MISC_FEATURE (2)..(3): x = (Aminoethyl)-glycine
  MISC_FEATURE (5)..(6): x = (Aminoethyl)-glycine
  MISC_FEATURE (8)..(9): x = (Aminoethyl)-glycine
  MISC_FEATURE (11)..(12): x = (Aminoethyl)-glycine
  MISC_FEATURE (14)..(15): x = (Aminoethyl)-glycine
  MISC_FEATURE (17)..(18): x = (Aminoethyl)-glycine
  MISC_FEATURE (20)..(21): x = (Aminoethyl)-glycine
  MISC_FEATURE (23)..(24): x = (Aminoethyl)-glycine
  MISC_FEATURE (26)..(27): x = peptide nucleic acid (thymine)
  MISC_FEATURE (29)..(30): x = peptide nucleic acid (thymine)
  MISC_FEATURE (32)..(33): x = peptide nucleic acid (thymine)
  MISC_FEATURE (35)..(36): x = (Aminoethyl)-glycine
  MISC_FEATURE (41)..(41): Carboxy terminus optionally may be converted to amide
XXXPXXPXXPXXPXXPXXPXXPXXPXXPXXPXXPXXPKKKK

SEQ ID NO: 206 - protein, 47 aa, Artificial Sequence
  Polymer tag
  MISC_FEATURE (1)..(1): x = 4-nitrophenylalanine
  MISC_FEATURE (2)..(3): x = epsilon-linked lysine
  MISC_FEATURE (5)..(6): x = epsilon-linked lysine
  MISC_FEATURE (8)..(9): x = epsilon-linked lysine
  MISC_FEATURE (11)..(12): x = epsilon-linked lysine
  MISC_FEATURE (14)..(15): x = epsilon-linked lysine
  MISC_FEATURE (17)..(18): x = epsilon-linked lysine
  MISC_FEATURE (20)..(21): x = epsilon-linked lysine
  MISC_FEATURE (23)..(24): x = epsilon-linked lysine
  MISC_FEATURE (26)..(29): x = Lysine-Peg4
  MISC_FEATURE (31)..(34): x = Lysine-Peg4
  MISC_FEATURE (36)..(39): x = Lysine-Peg4
  MISC_FEATURE (41)..(42): x = epsilon-linked lysine
  MISC_FEATURE (47)..(47): Carboxy terminus optionally may be converted to amide
XXXPXXPXXPXXPXXPXXPXXPXXPXXXXPXXXXPXXXXPXXPKKKK

SEQ ID NO: 207 - protein, 47 aa, Artificial Sequence
  Polymer tag
  MISC_FEATURE (1)..(1): x = 4-nitrophenylalanine
  MISC_FEATURE (2)..(3): x = epsilon-linked lysine
  MISC_FEATURE (5)..(6): x = epsilon-linked lysine
  MISC_FEATURE (8)..(9): x = epsilon-linked lysine
  MISC_FEATURE (11)..(12): x = epsilon-linked lysine
  MISC_FEATURE (14)..(15): x = epsilon-linked lysine
  MISC_FEATURE (17)..(18): x = epsilon-linked lysine
  MISC_FEATURE (20)..(21): x = epsilon-linked lysine
  MISC_FEATURE (23)..(24): x = epsilon-linked lysine
  MISC_FEATURE (27)..(27): x = lysine-PEG
  MISC_FEATURE (29)..(29): x = lysine-PEG
  MISC_FEATURE (32)..(32): x = lysine-PEG
  MISC_FEATURE (34)..(34): x = lysine-PEG
  MISC_FEATURE (37)..(37): x = lysine-PEG
  MISC_FEATURE (39)..(39): x = lysine-PEG
  MISC_FEATURE (41)..(42): x = epsilon-linked lysine
  MISC_FEATURE (47)..(47): Carboxy terminus optionally may be converted to amide
XXXPXXPXXPXXPXXPXXPXXPXXPGXGXPGXGXPGXGXPXXPKKKK

SEQ ID NO: 208 - protein, 41 aa, Artificial Sequence; identical to SEQ ID NO: 205
  Polymer tag
  MISC_FEATURE (1)..(1): x = 4-nitrophenylalanine
  MISC_FEATURE (2)..(3): x = epsilon-linked lysine
  MISC_FEATURE (5)..(6): x = epsilon-linked lysine
  MISC_FEATURE (8)..(9): x = epsilon-linked lysine
  MISC_FEATURE (11)..(12): x = epsilon-linked lysine
  MISC_FEATURE (14)..(15): x = epsilon-linked lysine
  MISC_FEATURE (17)..(18): x = epsilon-linked lysine
  MISC_FEATURE (20)..(21): x = epsilon-linked lysine
  MISC_FEATURE (23)..(24): x = peptide nucleic acid (thymine)
  MISC_FEATURE (26)..(27): x = peptide nucleic acid (thymine)
  MISC_FEATURE (29)..(30): x = peptide nucleic acid (thymine)
  MISC_FEATURE (32)..(33): x = peptide nucleic acid (thymine)
  MISC_FEATURE (35)..(36): x = epsilon-linked lysine
  MISC_FEATURE (41)..(41): Carboxy terminus optionally may be converted to amide

SEQ ID NO: 209 - protein, 41 aa, Artificial Sequence; identical to SEQ ID NO: 205
  Polymer tag
  MISC_FEATURE (1)..(1): x = 4-nitrophenylalanine
  MISC_FEATURE (2)..(3): x = epsilon-linked lysine
  MISC_FEATURE (5)..(6): x = epsilon-linked lysine
  MISC_FEATURE (8)..(9): x = epsilon-linked lysine
  MISC_FEATURE (11)..(12): x = epsilon-linked lysine
  MISC_FEATURE (14)..(15): x = epsilon-linked lysine
  MISC_FEATURE (17)..(18): x = epsilon-linked lysine
  MISC_FEATURE (20)..(21): x = epsilon-linked lysine
  MISC_FEATURE (23)..(24): x = epsilon-linked lysine
  MISC_FEATURE (26)..(27): x = peptide nucleic acid (thymine)
  MISC_FEATURE (29)..(30): x = peptide nucleic acid (thymine)
  MISC_FEATURE (32)..(33): x = peptide nucleic acid (thymine)
  MISC_FEATURE (35)..(36): x = epsilon-linked lysine
  MISC_FEATURE (41)..(41): Carboxy terminus optionally may be converted to amide

SEQ ID NO: 210 - protein, 47 aa, Artificial Sequence
  Polymer tag
  MISC_FEATURE (1)..(1): 4-nitrophenylalanine
  MISC_FEATURE (2)..(3): x = epsilon-linked lysine
  MISC_FEATURE (5)..(6): x = epsilon-linked lysine
  MISC_FEATURE (8)..(9): x = epsilon-linked lysine
  MISC_FEATURE (11)..(12): x = epsilon-linked lysine
  MISC_FEATURE (14)..(15): x = epsilon-linked lysine
  MISC_FEATURE (17)..(18): x = epsilon-linked lysine
  MISC_FEATURE (20)..(21): x = epsilon-linked lysine
  MISC_FEATURE (23)..(24): x = epsilon-linked lysine
  MISC_FEATURE (26)..(27): x = peptide nucleic acid (thymine)
  MISC_FEATURE (29)..(30): x = peptide nucleic acid (thymine)
  MISC_FEATURE (32)..(33): x = peptide nucleic acid (thymine)
  MISC_FEATURE (35)..(36): x = epsilon-linked lysine
  MISC_FEATURE (38)..(39): x = epsilon-linked lysine
  MISC_FEATURE (41)..(42): x = epsilon-linked lysine
  MISC_FEATURE (47)..(47): Carboxy terminus optionally may be converted to amide
XXXPXXPXXPXXPXXPXXPXXPXXPXXPXXPXXPXXPXXPXXPKKKK

SEQ ID NO: 211 - protein, 41 aa, Artificial Sequence
  Polymer tag
  MISC_FEATURE (1)..(1): x = hexynyl-4-nitrophenylalanine
  MISC_FEATURE (2)..(3): x = (Aminoethyl)-glycine
  MISC_FEATURE (5)..(6): x = (Aminoethyl)-glycine
  MISC_FEATURE (8)..(9): x = (Aminoethyl)-glycine
  MISC_FEATURE (11)..(12): x = (Aminoethyl)-glycine
  MISC_FEATURE (14)..(15): x = (Aminoethyl)-glycine
  MISC_FEATURE (17)..(18): x = (Aminoethyl)-glycine
  MISC_FEATURE (20)..(21): x = peptide nucleic acid (thymine)
  MISC_FEATURE (23)..(24): x = peptide nucleic acid (thymine)
  MISC_FEATURE (26)..(27): x = peptide nucleic acid (thymine)
  MISC_FEATURE (29)..(30): x = (Aminoethyl)-glycine
  MISC_FEATURE (32)..(33): x = (Aminoethyl)-glycine
  MISC_FEATURE (35)..(36): x = (Aminoethyl)-glycine
  MISC_FEATURE (41)..(41): Carboxy terminus optionally may be converted to amide
XXXGXXGXXGXXGXXGXXGXXPXXPXXPXXGXXGXXGKKKK

SEQ ID NO: 212 - protein, 41 aa, Artificial Sequence; identical to SEQ ID NO: 211
  Polymer tag
  MISC_FEATURE (1)..(1): x = hexynyl-4-nitrophenylalanine
  MISC_FEATURE (2)..(3): x = (Aminoethyl)-glycine
  MISC_FEATURE (5)..(6): x = (Aminoethyl)-glycine
  MISC_FEATURE (8)..(9): x = (Aminoethyl)-glycine
  MISC_FEATURE (11)..(12): x = (Aminoethyl)-glycine
  MISC_FEATURE (14)..(15): x = (Aminoethyl)-glycine
  MISC_FEATURE (17)..(18): x = (Aminoethyl)-glycine
  MISC_FEATURE (20)..(21): x = peptide nucleic acid (thymine)
  MISC_FEATURE (23)..(24): x = peptide nucleic acid (thymine)
  MISC_FEATURE (26)..(27): x = peptide nucleic acid (thymine)
  MISC_FEATURE (29)..(30): x = (Aminoethyl)-glycine
  MISC_FEATURE (32)..(33): x = (Aminoethyl)-glycine
  MISC_FEATURE (35)..(36): x = (Aminoethyl)-glycine
  MISC_FEATURE (41)..(41): Carboxy terminus optionally may be converted to amide

SEQ ID NO: 213 - protein, 47 aa, Artificial Sequence; identical to SEQ ID NO: 207
  Polymer tag
  MISC_FEATURE (1)..(1): x = hexynyl-4-nitrophenylalanine
  MISC_FEATURE (2)..(3): x = (aminoethyl)-glycine
  MISC_FEATURE (5)..(6): x = (aminoethyl)-glycine
  MISC_FEATURE (8)..(9): x = (aminoethyl)-glycine
  MISC_FEATURE (11)..(12): x = (aminoethyl)-glycine
  MISC_FEATURE (14)..(15): x = (aminoethyl)-glycine
  MISC_FEATURE (17)..(18): x = (aminoethyl)-glycine
  MISC_FEATURE (20)..(21): x = (aminoethyl)-glycine
  MISC_FEATURE (23)..(24): x = (aminoethyl)-glycine
  MISC_FEATURE (27)..(27): x = lysine-PEG4
  MISC_FEATURE (29)..(29): x = lysine-PEG4
  MISC_FEATURE (32)..(32): x = lysine-PEG4
  MISC_FEATURE (34)..(34): x = lysine-PEG4
  MISC_FEATURE (37)..(37): x = lysine-PEG4
  MISC_FEATURE (39)..(39): x = lysine-PEG4
  MISC_FEATURE (41)..(42): x = (aminoethyl)-glycine
  MISC_FEATURE (47)..(47): Carboxy terminus optionally may be converted to amide

SEQ ID NO: 214 - protein, 48 aa, Artificial Sequence
  Polymer tag
  MISC_FEATURE (1)..(1): x = hexynyl-4-nitrophenylalanine
  MISC_FEATURE (2)..(3): x = (aminoethyl)-glycine
  MISC_FEATURE (5)..(6): x = (aminoethyl)-glycine
  MISC_FEATURE (8)..(9): x = (aminoethyl)-glycine
  MISC_FEATURE (11)..(12): x = (aminoethyl)-glycine
  MISC_FEATURE (14)..(15): x = (aminoethyl)-glycine
  MISC_FEATURE (17)..(18): x = (aminoethyl)-glycine
  MISC_FEATURE (20)..(21): x = (aminoethyl)-glycine
  MISC_FEATURE (23)..(24): x = (aminoethyl)-glycine
  MISC_FEATURE (26)..(26): x = lysine-PEG
  MISC_FEATURE (28)..(28): x = lysine-PEG
  MISC_FEATURE (30)..(30): x = lysine-PEG
  MISC_FEATURE (32)..(32): x = lysine-PEG
  MISC_FEATURE (34)..(34): x = lysine-PEG
  MISC_FEATURE (36)..(36): x = lysine-PEG
  MISC_FEATURE (38)..(38): x = lysine-PEG
  MISC_FEATURE (40)..(40): x = lysine-PEG
  MISC_FEATURE (42)..(43): x = (aminoethyl)-glycine
  MISC_FEATURE (48)..(48): Carboxy terminus optionally may be converted to amide
XXXPXXPXXPXXPXXPXXPXXPXXPXGXGXGXGXGXGXGXGXXPKKKK

SEQ ID NO: 215 - protein, 41 aa, Artificial Sequence; identical to SEQ ID NO: 205
  Polymer tag
  MISC_FEATURE (1)..(1): x = hexynyl-4-nitrophenylalanine
  MISC_FEATURE (2)..(3): x = (aminoethyl)-glycine
  MISC_FEATURE (5)..(6): x = (aminoethyl)-glycine
  MISC_FEATURE (8)..(9): x = (aminoethyl)-glycine
  MISC_FEATURE (11)..(12): x = (aminoethyl)-glycine
  MISC_FEATURE (14)..(15): x = (aminoethyl)-glycine
  MISC_FEATURE (17)..(18): x = (aminoethyl)-glycine
  MISC_FEATURE (20)..(21): x = (aminoethyl)-glycine
  MISC_FEATURE (23)..(24): x = peptide nucleic acid (thymine)
  MISC_FEATURE (26)..(27): x = peptide nucleic acid (thymine)
  MISC_FEATURE (29)..(30): x = peptide nucleic acid (thymine)
  MISC_FEATURE (32)..(33): x = peptide nucleic acid (thymine)
  MISC_FEATURE (35)..(36): x = (aminoethyl)-glycine
  MISC_FEATURE (41)..(41): Carboxy terminus optionally may be converted to amide

SEQ ID NO: 216 - protein, 38 aa, Artificial Sequence
  Polymer tag
  MISC_FEATURE (1)..(1): x = hexynyl-4-nitrophenylalanine
  MISC_FEATURE (2)..(3): x = (aminoethyl)-glycine
  MISC_FEATURE (5)..(6): x = (aminoethyl)-glycine
  MISC_FEATURE (8)..(9): x = (aminoethyl)-glycine
  MISC_FEATURE (11)..(12): x = (aminoethyl)-glycine
  MISC_FEATURE (14)..(15): x = (aminoethyl)-glycine
  MISC_FEATURE (17)..(18): x = (aminoethyl)-glycine
  MISC_FEATURE (20)..(21): x = (aminoethyl)-glycine
  MISC_FEATURE (23)..(24): x = (aminoethyl)-glycine
  MISC_FEATURE (26)..(26): x = (aminoethyl)-glycine
  MISC_FEATURE (27)..(29): x = peptide nucleic acid (thymine)
  MISC_FEATURE (30)..(30): x = (aminoethyl)-glycine
  MISC_FEATURE (31)..(33): x = peptide nucleic acid (thymine)
  MISC_FEATURE (34)..(34): x = (aminoethyl)-glycine
  MISC_FEATURE (38)..(38): Carboxy terminus optionally may be converted to amide
XXXPXXPXXPXXPXXPXXPXXPXXPXXXXXXXXXKKKK

SEQ ID NO: 217 - protein, 8 aa, Artificial Sequence
  Polymer tag
  MISC_FEATURE (1)..(1): x = hexynyl-4-nitrophenylalanine
  MISC_FEATURE (2)..(2): x = polyethylene glycol 24mer
  MISC_FEATURE (3)..(4): x = epsilon-linked lysine
  MISC_FEATURE (8)..(8): Carboxy terminus optionally may be converted to amide
XXXXKKKK

SEQ ID NO: 218 - protein, 47 aa, Artificial Sequence; identical to SEQ ID NO: 207
  Polymer tag
  MISC_FEATURE (1)..(1): x = hexynyl-4-nitrophenylalanine
  MISC_FEATURE (2)..(3): x = (aminoethyl)-glycine
  MISC_FEATURE (5)..(6): x = (aminoethyl)-glycine
  MISC_FEATURE (8)..(9): x = (aminoethyl)-glycine
  MISC_FEATURE (11)..(12): x = (aminoethyl)-glycine
  MISC_FEATURE (14)..(15): x = (aminoethyl)-glycine
  MISC_FEATURE (17)..(18): x = (aminoethyl)-glycine
  MISC_FEATURE (20)..(21): x = (aminoethyl)-glycine
  MISC_FEATURE (23)..(24): x = (aminoethyl)-glycine
  MISC_FEATURE (27)..(27): x = lysine-PEG3
  MISC_FEATURE (29)..(29): x = lysine-PEG3
  MISC_FEATURE (32)..(32): x = lysine-PEG3
  MISC_FEATURE (34)..(34): x = lysine-PEG3
  MISC_FEATURE (37)..(37): x = lysine-PEG3
  MISC_FEATURE (39)..(39): x = lysine-PEG3
  MISC_FEATURE (41)..(42): x = (aminoethyl)-glycine
  MISC_FEATURE (47)..(47): Carboxy terminus optionally may be converted to amide

SEQ ID NO: 219 - protein, 49 aa, Artificial Sequence
  Polymer tag
  MISC_FEATURE (1)..(1): x = hexynyl-4-nitrophenylalanine
  MISC_FEATURE (2)..(3): x = (aminoethyl)-glycine
  MISC_FEATURE (5)..(6): x = (aminoethyl)-glycine
  MISC_FEATURE (8)..(9): x = (aminoethyl)-glycine
  MISC_FEATURE (11)..(12): x = (aminoethyl)-glycine
  MISC_FEATURE (14)..(15): x = (aminoethyl)-glycine
  MISC_FEATURE (17)..(18): x = (aminoethyl)-glycine
  MISC_FEATURE (20)..(21): x = (aminoethyl)-glycine
  MISC_FEATURE (24)..(24): x = lysine-PEG3
  MISC_FEATURE (26)..(26): x = lysine-PEG3
  MISC_FEATURE (29)..(29): x = lysine-PEG3
  MISC_FEATURE (31)..(31): x = lysine-PEG3
  MISC_FEATURE (34)..(34): x = lysine-PEG3
  MISC_FEATURE (36)..(36): x = lysine-PEG3
  MISC_FEATURE (39)..(39): x = lysine-PEG3
  MISC_FEATURE (41)..(41): x = lysine-PEG3
  MISC_FEATURE (43)..(44): x = (aminoethyl)-glycine
  MISC_FEATURE (49)..(49): Carboxy terminus optionally may be converted to amide
XXXPXXPXXPXXPXXPXXPXXPGXGXPGXGXPGXGXPGXGXPXXPKKKK

SEQ ID NO: 220 - protein, 41 aa, Artificial Sequence; identical to SEQ ID NO: 205
  Polymer tag
  MISC_FEATURE (1)..(1): x = hexynyl-4-nitrophenylalanine
  MISC_FEATURE (2)..(3): x = (aminoethyl)-glycine
  MISC_FEATURE (5)..(6): x = (aminoethyl)-glycine
  MISC_FEATURE (8)..(9): x = (aminoethyl)-glycine
  MISC_FEATURE (11)..(12): x = (aminoethyl)-glycine
  MISC_FEATURE (14)..(15): x = (aminoethyl)-glycine
  MISC_FEATURE (17)..(18): x = (aminoethyl)-glycine
  MISC_FEATURE (20)..(21): x = (aminoethyl)-glycine
  MISC_FEATURE (23)..(24): x = (aminoethyl)-glycine
  MISC_FEATURE (26)..(27): x = Aminoethylglycine-Peg4
  MISC_FEATURE (29)..(30): x = Aminoethylglycine-Peg4
  MISC_FEATURE (32)..(33): x = Aminoethylglycine-Peg4
  MISC_FEATURE (35)..(36): x = (aminoethyl)-glycine
  MISC_FEATURE (41)..(41): Carboxy terminus optionally may be converted to amide

SEQ ID NO: 221 - protein, 41 aa, Artificial Sequence; identical to SEQ ID NO: 205
  Polymer tag
  MISC_FEATURE (1)..(1): x = hexynyl-4-nitrophenylalanine
  MISC_FEATURE (2)..(3): x = (aminoethyl)-glycine
  MISC_FEATURE (5)..(6): x = (aminoethyl)-glycine
  MISC_FEATURE (8)..(9): x = (aminoethyl)-glycine
  MISC_FEATURE (11)..(12): x = (aminoethyl)-glycine
  MISC_FEATURE (14)..(15): x = (aminoethyl)-glycine
  MISC_FEATURE (17)..(18): x = (aminoethyl)-glycine
  MISC_FEATURE (20)..(21): x = (aminoethyl)-glycine
  MISC_FEATURE (23)..(24): x = (aminoethyl)-glycine
  MISC_FEATURE (26)..(27): x = peptide nucleic acid (cytosine)
  MISC_FEATURE (29)..(30): x = peptide nucleic acid (cytosine)
  MISC_FEATURE (32)..(33): x = peptide nucleic acid (cytosine)
  MISC_FEATURE (35)..(36): x = (aminoethyl)-glycine
  MISC_FEATURE (41)..(41): Carboxy terminus optionally may be converted to amide

SEQ ID NO: 222 - protein, 46 aa, Artificial Sequence
  Polymer tag
  MISC_FEATURE (1)..(1): x = hexynyl group
  MISC_FEATURE (46)..(46): Carboxy terminus optionally may be converted to amide
XKKKPPKKPPKKPPKKPPKKPPKKPPKKPPKKPPKKPPKKPPKKKK

SEQ ID NO: 223 - protein, 56 aa, Artificial Sequence
  Polymer tag
  MISC_FEATURE (1)..(1): x = hexynyl group
  MISC_FEATURE (56)..(56): Carboxy terminus optionally may be converted to amide
XKKKPPPKKPPPKKPPPKKPPPKKPPPKKPPPKKPPPKKPPPKKPPPKKPPPKKKK

SEQ ID NO: 224 - protein, 36 aa, Artificial Sequence
  Polymer tag
  MISC_FEATURE (1)..(1): x = hexynyl group
  MISC_FEATURE (2)..(4): x = epsilon-linked lysine
  MISC_FEATURE (6)..(7): x = epsilon-linked lysine
  MISC_FEATURE (9)..(10): x = epsilon-linked lysine
  MISC_FEATURE (12)..(13): x = epsilon-linked lysine
  MISC_FEATURE (15)..(16): x = epsilon-linked lysine
  MISC_FEATURE (18)..(19): x = epsilon-linked lysine
  MISC_FEATURE (21)..(22): x = epsilon-linked lysine
  MISC_FEATURE (24)..(25): x = epsilon-linked lysine
  MISC_FEATURE (27)..(28): x = epsilon-linked lysine
  MISC_FEATURE (30)..(31): x = epsilon-linked lysine
  MISC_FEATURE (36)..(36): Carboxy terminus optionally may be converted to amide
XXXXPXXPXXPXXPXXPXXPXXPXXPXXPXXPKKKK

SEQ ID NO: 225 - protein, 35 aa, Artificial Sequence; identical to SEQ ID NO: 170
  Polymer tag
  MISC_FEATURE (1)..(1): x = hexynyl-4-nitrophenylalanine
  MISC_FEATURE (2)..(3): x = epsilon-linked lysine
  MISC_FEATURE (5)..(6): x = epsilon-linked lysine
  MISC_FEATURE (8)..(9): x = epsilon-linked lysine
  MISC_FEATURE (11)..(12): x = epsilon-linked lysine
  MISC_FEATURE (14)..(15): x = epsilon-linked lysine
  MISC_FEATURE (17)..(18): x = epsilon-linked lysine
  MISC_FEATURE (20)..(21): x = epsilon-linked lysine
  MISC_FEATURE (23)..(24): x = epsilon-linked lysine
  MISC_FEATURE (26)..(27): x = epsilon-linked lysine
  MISC_FEATURE (29)..(30): x = epsilon-linked lysine
  MISC_FEATURE (35)..(35): Carboxy terminus optionally may be converted to amide

SEQ ID NO: 226 - protein, 45 aa, Artificial Sequence
  Polymer tag
  MISC_FEATURE (1)..(1): x = hexynyl-4-nitrophenylalanine
  MISC_FEATURE (2)..(2): beta-alanine
  MISC_FEATURE (4)..(4): beta-alanine
  MISC_FEATURE (6)..(6): beta-alanine
  MISC_FEATURE (8)..(8): beta-alanine
  MISC_FEATURE (10)..(10): beta-alanine
  MISC_FEATURE (12)..(12): beta-alanine
  MISC_FEATURE (14)..(14): beta-alanine
  MISC_FEATURE (16)..(16): beta-alanine
  MISC_FEATURE (18)..(18): beta-alanine
  MISC_FEATURE (20)..(20): beta-alanine
  MISC_FEATURE (22)..(22): beta-alanine
  MISC_FEATURE (24)..(24): beta-alanine
  MISC_FEATURE (26)..(26): beta-alanine
  MISC_FEATURE (28)..(28): beta-alanine
  MISC_FEATURE (30)..(30): beta-alanine
  MISC_FEATURE (32)..(32): beta-alanine
  MISC_FEATURE (34)..(34): beta-alanine
  MISC_FEATURE (36)..(36): beta-alanine
  MISC_FEATURE (38)..(38): beta-alanine
  MISC_FEATURE (40)..(40): beta-alanine
  MISC_FEATURE (45)..(45): Carboxy terminus optionally may be converted to amide
XAKAKAKAKAKAKAKAKAKAKAKAKAKAKAKAKAKAKAKAKKKKK

SEQ ID NO: 227 - protein, 45 aa, Artificial Sequence; identical to SEQ ID NO: 171
  Polymer tag
  MISC_FEATURE (1)..(1): x = hexynyl-epsilon-linked lysine
  MISC_FEATURE (2)..(3): x = (aminoethyl)-glycine
  MISC_FEATURE (6)..(7): x = (aminoethyl)-glycine
  MISC_FEATURE (10)..(11): x = (aminoethyl)-glycine
  MISC_FEATURE (14)..(15): x = (aminoethyl)-glycine
  MISC_FEATURE (18)..(19): x = (aminoethyl)-glycine
  MISC_FEATURE (22)..(23): x = (aminoethyl)-glycine
  MISC_FEATURE (26)..(27): x = (aminoethyl)-glycine
  MISC_FEATURE (30)..(31): x = (aminoethyl)-glycine
  MISC_FEATURE (34)..(35): x = (aminoethyl)-glycine
  MISC_FEATURE (38)..(39): x = (aminoethyl)-glycine
  MISC_FEATURE (45)..(45): Carboxy terminus optionally may be converted to amide

SEQ ID NO: 228 - protein, 9 aa, Artificial Sequence
  Polymer tag
  MISC_FEATURE (1)..(1): x = hexynyl-4-nitrophenylalanine
  MISC_FEATURE (2)..(2): x = polyethylene glycol 24mer
  MISC_FEATURE (3)..(4): x = (aminoethyl)-glycine
  MISC_FEATURE (9)..(9): Carboxy terminus optionally may be converted to amide
XXXXPKKKK

SEQ ID NO: 229 - protein, 27 aa, Artificial Sequence
  Polymer tag
  MISC_FEATURE (1)..(1): x = hexynyl-4-nitrophenylalanine
  MISC_FEATURE (2)..(3): x = (aminoethyl)-glycine
  MISC_FEATURE (5)..(6): x = (aminoethyl)-glycine
  MISC_FEATURE (8)..(9): x = (aminoethyl)-glycine
  MISC_FEATURE (11)..(12): x = (aminoethyl)-glycine
  MISC_FEATURE (14)..(15): x = (aminoethyl)-glycine
  MISC_FEATURE (17)..(18): x = (aminoethyl)-glycine
  MISC_FEATURE (20)..(20): x = polyethylene glycol 12mer
  MISC_FEATURE (21)..(22): x = (aminoethyl)-glycine
XXXPXXPXXPXXPXXPXXPXXXPKKKK

SEQ ID NO: 230 - protein, 41 aa, Artificial Sequence; identical to SEQ ID NO: 205
  Polymer tag
  MISC_FEATURE (1)..(1): x = hexynyl-4-nitrophenylalanine
  MISC_FEATURE (2)..(2): x = (aminoethyl)-glycine
  MISC_FEATURE (3)..(3): x = Oxoaminohexanoic acid
  MISC_FEATURE (5)..(5): x = (aminoethyl)-glycine
  MISC_FEATURE (6)..(6): x = Oxoaminohexanoic acid
  MISC_FEATURE (8)..(8): x = (aminoethyl)-glycine
  MISC_FEATURE (9)..(9): x = Oxoaminohexanoic acid
  MISC_FEATURE (11)..(11): x = (aminoethyl)-glycine
  MISC_FEATURE (12)..(12): x = Oxoaminohexanoic acid
  MISC_FEATURE (14)..(14): x = (aminoethyl)-glycine
  MISC_FEATURE (15)..(15): x = Oxoaminohexanoic acid
  MISC_FEATURE (17)..(17): x = (aminoethyl)-glycine
  MISC_FEATURE (18)..(18): x = Oxoaminohexanoic acid
  MISC_FEATURE (20)..(20): x = (aminoethyl)-glycine
  MISC_FEATURE (21)..(21): x = Oxoaminohexanoic acid
  MISC_FEATURE (23)..(24): x = peptide nucleic acid (thymine)
  MISC_FEATURE (26)..(27): x = peptide nucleic acid (thymine)
  MISC_FEATURE (29)..(30): x = peptide nucleic acid (thymine)
  MISC_FEATURE (32)..(33): x = peptide nucleic acid (thymine)
  MISC_FEATURE (35)..(36): x = (aminoethyl)-glycine

SEQ ID NO: 231 - protein, 41 aa, Artificial Sequence; identical to SEQ ID NO: 205
  Polymer tag
  MISC_FEATURE (1)..(1): x = hexynyl-4-nitrophenylalanine
  MISC_FEATURE (2)..(2): x = (aminoethyl)-glycine
  MISC_FEATURE (3)..(3): x = oxoaminohexanoic acid
  MISC_FEATURE (5)..(5): x = (aminoethyl)-glycine
  MISC_FEATURE (6)..(6): x = oxoaminohexanoic acid
  MISC_FEATURE (8)..(8): x = (aminoethyl)-glycine
  MISC_FEATURE (9)..(9): x = oxoaminohexanoic acid
  MISC_FEATURE (11)..(11): x = (aminoethyl)-glycine
  MISC_FEATURE (12)..(12): x = oxoaminohexanoic acid
  MISC_FEATURE (14)..(15): x = (aminoethyl)-glycine
  MISC_FEATURE (17)..(18): x = (aminoethyl)-glycine
  MISC_FEATURE (20)..(21): x = (aminoethyl)-glycine
  MISC_FEATURE (23)..(24): x = peptide nucleic acid (thymine)
  MISC_FEATURE (26)..(27): x = peptide nucleic acid (thymine)
  MISC_FEATURE (29)..(30): x = peptide nucleic acid (thymine)
  MISC_FEATURE (32)..(33): x = peptide nucleic acid (thymine)
  MISC_FEATURE (35)..(36): x = (aminoethyl)-glycine

SEQ ID NO: 232 - protein, 41 aa, Artificial Sequence; identical to SEQ ID NO: 205
  Polymer tag
  MISC_FEATURE (1)..(1): x = hexynyl-4-nitrophenylalanine
  MISC_FEATURE (2)..(3): x = (aminoethyl)-glycine
  MISC_FEATURE (5)..(6): x = (aminoethyl)-glycine
  MISC_FEATURE (8)..(9): x = (aminoethyl)-glycine
  MISC_FEATURE (11)..(11): x = (aminoethyl)-glycine
  MISC_FEATURE (12)..(12): x = oxoaminohexanoic acid
  MISC_FEATURE (14)..(14): x = (aminoethyl)-glycine
  MISC_FEATURE (15)..(15): x = oxoaminohexanoic acid
  MISC_FEATURE (17)..(17): x = (aminoethyl)-glycine
  MISC_FEATURE (18)..(18): x = oxoaminohexanoic acid
  MISC_FEATURE (20)..(20): x = (aminoethyl)-glycine
  MISC_FEATURE (21)..(21): x = oxoaminohexanoic acid
  MISC_FEATURE (23)..(24): x = peptide nucleic acid (thymine)
  MISC_FEATURE (26)..(27): x = peptide nucleic acid (thymine)
  MISC_FEATURE (29)..(30): x = peptide nucleic acid (thymine)
  MISC_FEATURE (32)..(33): x = peptide nucleic acid (thymine)
  MISC_FEATURE (35)..(36): x = (aminoethyl)-glycine

SEQ ID NO: 233 - protein, 41 aa, Artificial Sequence; identical to SEQ ID NO: 205
  Polymer tag
  MISC_FEATURE (1)..(1): x = hexynyl-4-nitrophenylalanine
  MISC_FEATURE (2)..(3): x = (aminoethyl)-glycine
  MISC_FEATURE (5)..(6): x = (aminoethyl)-glycine
  MISC_FEATURE (8)..(9): x = (aminoethyl)-glycine
  MISC_FEATURE (11)..(12): x = (aminoethyl)-glycine
  MISC_FEATURE (14)..(15): x = (aminoethyl)-glycine
  MISC_FEATURE (17)..(17): x = (aminoethyl)-glycine
  MISC_FEATURE (18)..(18): x = oxoaminohexanoic acid
  MISC_FEATURE (20)..(20): x = (aminoethyl)-glycine
  MISC_FEATURE (21)..(21): x = oxoaminohexanoic acid
  MISC_FEATURE (23)..(24): x = peptide nucleic acid (thymine)
  MISC_FEATURE (26)..(27): x = peptide nucleic acid (thymine)
  MISC_FEATURE (29)..(30): x = peptide nucleic acid (thymine)
  MISC_FEATURE (32)..(33): x = peptide nucleic acid (thymine)
  MISC_FEATURE (35)..(36): x = (aminoethyl)-glycine

SEQ ID NO: 234 - protein, 38 aa, Artificial Sequence
  Polymer tag
  MISC_FEATURE (1)..(1): x = hexynyl-4-nitrophenylalanine
  MISC_FEATURE (2)..(2): x = (aminoethyl)-glycine
  MISC_FEATURE (5)..(5): x = (aminoethyl)-glycine
  MISC_FEATURE (8)..(8): x = (aminoethyl)-glycine
  MISC_FEATURE (11)..(11): x = (aminoethyl)-glycine
  MISC_FEATURE (14)..(14): x = (aminoethyl)-glycine
  MISC_FEATURE (17)..(17): x = (aminoethyl)-glycine
  MISC_FEATURE (20)..(20): x = (aminoethyl)-glycine
  MISC_FEATURE (23)..(23): x = (aminoethyl)-glycine
  MISC_FEATURE (26)..(26): x = (aminoethyl)-glycine
  MISC_FEATURE (29)..(29): x = (aminoethyl)-glycine
  MISC_FEATURE (32)..(32): x = (aminoethyl)-glycine
XXGGXGGXGGXGGXGGXGGXGGXGGXGGXGGXGGKKKK

SEQ ID NO: 235 - protein, 38 aa, Artificial Sequence
  Polymer tag
  MISC_FEATURE (1)..(1): x = hexynyl-4-nitrophenylalanine
  MISC_FEATURE (2)..(2): x = (aminoethyl)-glycine
  MISC_FEATURE (5)..(5): x = (aminoethyl)-glycine
  MISC_FEATURE (8)..(8): x = (aminoethyl)-glycine
  MISC_FEATURE (11)..(11): x = (aminoethyl)-glycine
  MISC_FEATURE (14)..(14): x = (aminoethyl)-glycine
  MISC_FEATURE (17)..(17): x = (aminoethyl)-glycine
  MISC_FEATURE (20)..(20): x = (aminoethyl)-glycine
  MISC_FEATURE (23)..(23): x = (aminoethyl)-glycine
  MISC_FEATURE (26)..(26): x = (aminoethyl)-glycine
  MISC_FEATURE (29)..(29): x = (aminoethyl)-glycine
  MISC_FEATURE (32)..(32): x = (aminoethyl)-glycine
XXKPXKPXKPXKPXKPXKPXKPXKPXKPXKPXKPKKKK

SEQ ID NO: 236 - protein, 38 aa, Artificial Sequence
  Polymer tag
  MISC_FEATURE (1)..(1): x = hexynyl-4-nitrophenylalanine
  MISC_FEATURE (2)..(2): x = (aminoethyl)-glycine
  MISC_FEATURE (4)..(4): x = 4-benzyloxy proline
  MISC_FEATURE (5)..(5): x = (aminoethyl)-glycine
  MISC_FEATURE (7)..(7): x = 4-benzyloxy proline
  MISC_FEATURE (8)..(8): x = (aminoethyl)-glycine
  MISC_FEATURE (10)..(10): x = 4-benzyloxy proline
  MISC_FEATURE (11)..(11): x = (aminoethyl)-glycine
  MISC_FEATURE (13)..(13): x = 4-benzyloxy proline
  MISC_FEATURE (14)..(14): x = (aminoethyl)-glycine
  MISC_FEATURE (16)..(16): x = 4-benzyloxy proline
  MISC_FEATURE (17)..(17): x = (aminoethyl)-glycine
  MISC_FEATURE (19)..(19): x = 4-benzyloxy proline
  MISC_FEATURE (20)..(20): x = (aminoethyl)-glycine
  MISC_FEATURE (22)..(22): x = 4-benzyloxy proline
  MISC_FEATURE (23)..(23): x = (aminoethyl)-glycine
  MISC_FEATURE (25)..(25): x = 4-benzyloxy proline
  MISC_FEATURE (26)..(26): x = (aminoethyl)-glycine
  MISC_FEATURE (28)..(28): x = 4-benzyloxy proline
  MISC_FEATURE (29)..(29): x = (aminoethyl)-glycine
  MISC_FEATURE (31)..(31): x = 4-benzyloxy proline
  MISC_FEATURE (32)..(32): x = (aminoethyl)-glycine
  MISC_FEATURE (34)..(34): x = 4-benzyloxy proline
XXKXXKXXKXXKXXKXXKXXKXXKXXKXXKXXKXKKKK

SEQ ID NO: 237 - protein, 41 aa, Artificial Sequence
  Polymer tag
  MISC_FEATURE (1)..(1): x = hexynyl-4-nitrophenylalanine
  MISC_FEATURE (2)..(3): x = (aminoethyl)-glycine
  MISC_FEATURE (5)..(6): x = (aminoethyl)-glycine
  MISC_FEATURE (8)..(9): x = (aminoethyl)-glycine
  MISC_FEATURE (11)..(12): x = (aminoethyl)-glycine
  MISC_FEATURE (14)..(15): x = (aminoethyl)-glycine
  MISC_FEATURE (17)..(18): x = (aminoethyl)-glycine
  MISC_FEATURE (20)..(21): x = (aminoethyl)-glycine
  MISC_FEATURE (23)..(23): x = (aminoethyl)-glycine
  MISC_FEATURE (26)..(26): x = (aminoethyl)-glycine
  MISC_FEATURE (29)..(29): x = (aminoethyl)-glycine
  MISC_FEATURE (32)..(32): x = (aminoethyl)-glycine
  MISC_FEATURE (35)..(35): x = (aminoethyl)-glycine
XXXPXXPXXPXXPXXPXXPXXPXKPXKPXKPXKPXKPKKKK

SEQ ID NO: 238 - protein, 41 aa, Artificial Sequence; identical to SEQ ID NO: 205
  Polymer tag
  MISC_FEATURE (1)..(1): x = hexynyl-4-nitrophenylalanine
  MISC_FEATURE (2)..(3): x = (aminoethyl)-glycine
  MISC_FEATURE (5)..(6): x = (aminoethyl)-glycine
  MISC_FEATURE (8)..(9): x = (aminoethyl)-glycine
  MISC_FEATURE (11)..(12): x = (aminoethyl)-glycine
  MISC_FEATURE (14)..(15): x = (aminoethyl)-glycine
  MISC_FEATURE (17)..(18): x = (aminoethyl)-glycine
  MISC_FEATURE (20)..(21): x = (aminoethyl)-glycine
  MISC_FEATURE (23)..(23): x = Aminoethylglycine-Peg4
  MISC_FEATURE (24)..(24): x = (aminoethyl)-glycine
  MISC_FEATURE (26)..(26): x = Aminoethylglycine-Peg4
  MISC_FEATURE (27)..(27): x = (aminoethyl)-glycine
  MISC_FEATURE (29)..(29): x = Aminoethylglycine-Peg4
  MISC_FEATURE (30)..(30): x = (aminoethyl)-glycine
  MISC_FEATURE (32)..(32): x = Aminoethylglycine-Peg4
  MISC_FEATURE (33)..(33): x = (aminoethyl)-glycine
  MISC_FEATURE (35)..(36): x = (aminoethyl)-glycine

SEQ ID NO: 239 - protein, 41 aa, Artificial Sequence; identical to SEQ ID NO: 205
  Polymer tag
  MISC_FEATURE (1)..(1): x = hexynyl-4-nitrophenylalanine
  MISC_FEATURE (2)..(3): x = (aminoethyl)-glycine
  MISC_FEATURE (5)..(6): x = (aminoethyl)-glycine
  MISC_FEATURE (8)..(9): x = (aminoethyl)-glycine
  MISC_FEATURE (11)..(12): x = (aminoethyl)-glycine
  MISC_FEATURE (14)..(15): x = (aminoethyl)-glycine
  MISC_FEATURE (17)..(18): x = (aminoethyl)-glycine
  MISC_FEATURE (20)..(21): x = (aminoethyl)-glycine
  MISC_FEATURE (23)..(23): x = (aminoethyl)-glycine
  MISC_FEATURE (24)..(24): x = peptide nucleic acid (thymine)
  MISC_FEATURE (26)..(26): x = (aminoethyl)-glycine
  MISC_FEATURE (27)..(27): x = peptide nucleic acid (thymine)
  MISC_FEATURE (29)..(29): x = (aminoethyl)-glycine
  MISC_FEATURE (30)..(30): x = peptide nucleic acid (thymine)
  MISC_FEATURE (32)..(32): x = (aminoethyl)-glycine
  MISC_FEATURE (33)..(33): x = peptide nucleic acid (thymine)
  MISC_FEATURE (35)..(36): x = (aminoethyl)-glycine

SEQ ID NO: 240 - protein, 57 aa, Artificial Sequence
  Polymer tag
  MISC_FEATURE (1)..(1): x = hexynyl-4-nitrophenylalanine
  MISC_FEATURE (2)..(3): x = epsilon-linked lysine
  MISC_FEATURE (6)..(7): x = epsilon-linked lysine
  MISC_FEATURE (10)..(11): x = epsilon-linked lysine
  MISC_FEATURE (14)..(15): x = epsilon-linked lysine
  MISC_FEATURE (18)..(19): x = epsilon-linked lysine
  MISC_FEATURE (22)..(23): x = epsilon-linked lysine
  MISC_FEATURE (26)..(27): x = epsilon-linked lysine
  MISC_FEATURE (30)..(31): x = epsilon-linked lysine
  MISC_FEATURE (34)..(35): x = epsilon-linked lysine
  MISC_FEATURE (38)..(39): x = epsilon-linked lysine
  MISC_FEATURE (42)..(43): x = epsilon-linked lysine
  MISC_FEATURE (46)..(47): x = epsilon-linked lysine
  MISC_FEATURE (50)..(51): x = epsilon-linked lysine
XXXPPXXPPXXPPXXPPXXPPXXPPXXPPXXPPXXPPXXPPXXPPXXPPXXPPRRRR

SEQ ID NO: 241 - protein, 41 aa, Artificial Sequence; identical to SEQ ID NO: 205
  Polymer tag
  MISC_FEATURE (1)..(1): x = hexynyl-4-nitrophenylalanine
  MISC_FEATURE (2)..(3): x = (aminoethyl)-glycine
  MISC_FEATURE (5)..(6): x = (aminoethyl)-glycine
  MISC_FEATURE (8)..(9): x = (aminoethyl)-glycine
  MISC_FEATURE (11)..(12): x = (aminoethyl)-glycine
  MISC_FEATURE (14)..(15): x = (aminoethyl)-glycine
  MISC_FEATURE (17)..(18): x = (aminoethyl)-glycine
  MISC_FEATURE (20)..(21): x = (aminoethyl)-glycine
  MISC_FEATURE (23)..(24): x = (aminoethyl)-glycine
  MISC_FEATURE (26)..(27): x = (aminoethyl)-glycine
  MISC_FEATURE (29)..(30): x = (aminoethyl)-glycine
  MISC_FEATURE (32)..(33): x = (aminoethyl)-glycine
  MISC_FEATURE (35)..(36): x = (aminoethyl)-glycine

SEQ ID NO: 242 - protein, 41 aa, Artificial Sequence; identical to SEQ ID NO: 205
  Polymer tag
  MISC_FEATURE (1)..(1): x = hexynyl-4-nitrophenylalanine
  MISC_FEATURE (2)..(3): x = 4-Aminoproline
  MISC_FEATURE (5)..(6): x = 4-Aminoproline
  MISC_FEATURE (8)..(9): x = 4-Aminoproline
  MISC_FEATURE (11)..(12): x = 4-Aminoproline
  MISC_FEATURE (14)..(15): x = 4-Aminoproline
  MISC_FEATURE (17)..(18): x = 4-Aminoproline
  MISC_FEATURE (20)..(21): x = 4-Aminoproline
  MISC_FEATURE (23)..(24): x = 4-Aminoproline
  MISC_FEATURE (26)..(27): x = 4-Aminoproline
  MISC_FEATURE (29)..(30): x = 4-Aminoproline
  MISC_FEATURE (32)..(33): x = 4-Aminoproline
  MISC_FEATURE (35)..(36): x = 4-Aminoproline

SEQ ID NO: 243 - DNA, 30 bp, Artificial Sequence
  Sp2 Tag
  misc_feature (1)..(8): n = 2-carbon abasic site of Formula 8
  misc_feature (15)..(30): n = 2-carbon abasic site of Formula 8
nnnnnnnnttttttnnnnnnnnnnnnnnnn